European Patent Specification EP 3 894 429 B1, published February 21, 2024. Title: CRIMEAN-CONGO HEMORRHAGIC FEVER VIRUS REPLICON PARTICLES AND USE THEREOF. Applicant: UNIVERSITY OF GEORGIA RESEARCH FOUNDATION, INC. The sequence listing filed with the application follows.

SEQUENCE LISTING (22 sequences)

SEQ ID NO: 1 - DNA, 4576 bp, Artificial Sequence
  Synthetic construct (pT7-S)
gctgaaaggaggaactatatccggatcgagatcctctaggtacaagcctaattgtgtagcatctggcttactgaagcagaccctatcatctctctcgtaaactgccgtcagagtcggtttggttggacgaaccttctgagtttctggtaacgccgtcccgcacccggaaatggtcagcgaaccaatcagcagggtcatcgctagccagatcctctacgccggacgcatcgtggccggcatcaccggcgccacaggtgcggttgctggcgcctatatcgccgacatcaccgatggggaagatcgggctcgccacttcgggctcatgagcgcttgtttcggcgtgggtatggtggcaggccccgtggccgggggactgttgggcgccatctccttgcaccattccttgcggcggcggtgctcaacggcctcaacctactactgggctgcttcctaatgcaggagtcgcataagggagagcgtcgatatggtgcactctcagtacaatctgctctgatgccgcatagttaagccagccccgacacccgccaacacccgctgacgcgccctgacgggcttgtctgctcccggcatccgcttacagacaagctgtgacaaagggcctcgtgatacgcctatttttataggttaatgtcatgataataatggtttcttagacgtcaggtggcacttttcggggaaatgtgcgcggaacccctatttgtttatttttctaaatacattcaaatatgtatccgctcatgagacaataaccctgataaatgcttcaataatattgaaaaaggaagagtatgagtattcaacatttccgtgtcgcccttattcccttttttgcggcattttgccttcctgtttttgctcacccagaaacgctggtgaaagtaaaagatgctgaagatcagttgggtgcacgagtgggttacatcgaactggatctcaacagcggtaagatccttgagagttttcgccccgaagaacgttttccaatgatgagcacttttaaagttctgctatgtggcgcggtattatcccgtattgacgccgggcaagagcaactcggtcgccgcatacactattctcagaatgacttggttgagtactcaccagtcacagaaaagcatcttacggatggcatgacagtaagagaattatgcagtgctgccataaccatgagtgataacactgcggccaacttacttctgacaacgatcggaggaccgaaggagctaaccgcttttttgcacaacatgggggatcatgtaactcgccttgatcgttgggaaccggagctgaatgaagccataccaaacgacgagcgtgacaccacgatgcctgtagcaatggcaacaacgttgcgcaaactattaactggcgaactacttactctagcttcccggcaacaattaatagactggatggaggcggataaagttgcaggaccacttctgcgctcggcccttccggctggctggtttattgctgataaatctggagccggtgagcgtgggtctcgcggtatcattgcagcactggggccagatggtaagccctcccgtatcgtagttatctacacgacggggagtcaggcaactatggatgaacgaaatagacagatcgctgagataggtgcctcactgattaagcattggtaactgtcagaccaagtttactcatatatactttagattgatttaaaacttcatttttaatttaaaaggatctaggtgaagatcctttttgataatctcatgaccaaaatcccttaacgtgagttttcgttccactgagcgtcagaccccgtagaaaagatcaaaggatcttcttgagatcctttttttctgcgcgtaatctgctgcttgcaaacaaaaaaaccaccgctaccagcggtggtttgtttgccggatcaagagctaccaactctttttccgaaggtaactggcttcagcagagcgcagataccaaatactgtccttctagtgtagccgtagttaggccaccacttcaagaactctgtagcaccgcctacatacctcgctctgctaatcctgttaccagtggctgctgccagtggcgataagtcgtgtcttaccgggttggactcaagacgatagttaccggataaggcgcagcggtcgggctgaacggggggttcgtgcacacagcccagcttggagcgaacgacctacaccgaactgagatacctacagcgtgagctatgagaaagcgccacgcttcccgaagggagaaaggcggacaggtatccggtaagcggcagggtcggaacaggagagcgcacgagggagcttccagggggaaacgcctggtatctttatagtcctgtcgggtttcgccacctctgacttgagcgtcgatttttgtgatgctcgtcaggggggcggagcctatggaaaaacgccagcaacgcggcctttttacggttcctggccttttgctggccttttgctcacatgttctttcctgcgttatcccctgattctgtggataaccgtattaccgcctttgagtgagctgataccgctcgccgcagccgaacgaccgagcgcagcgagtcagtgagcgaggaagcggaagagcgcccaatacgcaaaccgcctctccccgcgcgttggccgattcattaatgcagggggatctcgatcccgcgaaattaatacgactcactatagtctcaaagaaacacgtgccgcttacgcccacagtgttctcttgagtgttagcagaatggaaaacaagatcgaggtgaataacaaagatgagatgaacaggtggtttgaagagttcaaaaaaggaaatggacttgtggacaccttcacaaactcctattccttttgcgagagtgttcccaatttggacaggtttgtgtttcagatggccagtgccaccgatgatgcacagaaggactccatctacgcatctgctctggtggaggcaacaaagttttgtgcacctatatatgagtgcgcatgggttagctccactggcattgtaaaaaagggacttgaatggttcgagaaaaatgcaggaaccattaagtcctgggatgaaagttatactgagctaaaggtcgacgtcccgaaaatagagcagcttaccggttaccaacaagctgccttgaagtggagaaaagacataggtttccgtgtcaatgccaacacagcagctctgagcaacaaagtcctcgcagaatacaaagtccctggtgagattgtgatgtctgtcaaagagatgctgtcagacatgattaggagaaggaacctgattctaaacaggggtggtgatgagaacccacgtggcccagtgagccatgagcatgtagactggtgcagggagtttgtcaaaggcaaatacatcatggccttcaacccaccatggggggacatcaacaagtcaggccgttcaggaatagcacttgttgcaacaggccttgctaagcttgcagagactgaaggaaagggaatatttgatgaagccaaaaagactgtggaggccctcaacgggtatctggacaagcataaggacgaagttgatagagcaagcgccgacagcatgataacaaaccttcttaagcatattgccaaggcacaggagctctataaaaattcatctgcacttcgtgcacaaagcgcacagattgacactgctttcagctcatactattggctttacaaggctggcgtgactcctgaaaccttcccgacggtgtcacagttcctctttgagctagggaaacagccaagaggtaccaagaaaatgaagaaggctcttctgagcaccccaatgaagtgggggaagaagctttatgagctctttgccgatgattctttccagcagaacaggatttacatgcatcctgccgtgcttacagctggtagaatcagtgaaatgggagtctgctttgggacaatccctgtggccaatcctgatgatgctgcccaaggatctggacacactaagtctattctcaacctccgtaccaacactgagaccaataatccgtgtgccaaaaccatcgtcaagctatttgaagttcaaaaaacagggttcaacattcaggacatggacatagtggcctctgagcacttgctacaccaatcccttgttggcaagcaatccccattccagaacgcctacaacgtcaagggcaatgccaccagtgctaacatcatttaaaatacaaactgctctgtactcaacttccttccttctgaaccgccatccataattgcaatacttaatcatgcttttttacttgcttatgtaaccttattttattaacctttctctattttctcttgttttaaacacttaaagggctgtgcggcaacgatatctttgagagggtcggcatggcatctccacctcctcgcggtccgacctgggcatccgaaggaggacgtcgtccactcggatggctaagggagagctcggatccggctgctaacaaagcccgaaaggaagctgagttggctgctgccaccgctgagcaataactagcataaccccttggggcctctaaacgggtcttgaggggtttttt

SEQ ID NO: 2 - DNA, 15064 bp, Artificial Sequence
  Synthetic construct (pT7-L)
gctgaaaggaggaactatatccggatcgagatcctctaggtacaagcctaattgtgtagcatctggcttactgaagcagaccctatcatctctctcgtaaactgccgtcagagtcggtttggttggacgaaccttctgagtttctggtaacgccgtcccgcacccggaaatggtcagcgaaccaatcagcagggtcatcgctagccagatcctctacgccggacgcatcgtggccggcatcaccggcgccacaggtgcggttgctggcgcctatatcgccgacatcaccgatggggaagatcgggctcgccacttcgggctcatgagcgcttgtttcggcgtgggtatggtggcaggccccgtggccgggggactgttgggcgccatctccttgcaccattccttgcggcggcggtgctcaacggcctcaacctactactgggctgcttcctaatgcaggagtcgcataagggagagcgtcgatatggtgcactctcagtacaatctgctctgatgccgcatagttaagccagccccgacacccgccaacacccgctgacgcgccctgacgggcttgtctgctcccggcatccgcttacagacaagctgtgacaaagggcctcgtgatacgcctatttttataggttaatgtcatgataataatggtttcttagacgtcaggtggcacttttcggggaaatgtgcgcggaacccctatttgtttatttttctaaatacattcaaatatgtatccgctcatgagacaataaccctgataaatgcttcaataatattgaaaaaggaagagtatgagtattcaacatttccgtgtcgcccttattcccttttttgcggcattttgccttcctgtttttgctcacccagaaacgctggtgaaagtaaaagatgctgaagatcagttgggtgcacgagtgggttacatcgaactggatctcaacagcggtaagatccttgagagttttcgccccgaagaacgttttccaatgatgagcacttttaaagttctgctatgtggcgcggtattatcccgtattgacgccgggcaagagcaactcggtcgccgcatacactattctcagaatgacttggttgagtactcaccagtcacagaaaagcatcttacggatggcatgacagtaagagaattatgcagtgctgccataaccatgagtgataacactgcggccaacttacttctgacaacgatcggaggaccgaaggagctaaccgcttttttgcacaacatgggggatcatgtaactcgccttgatcgttgggaaccggagctgaatgaagccataccaaacgacgagcgtgacaccacgatgcctgtagcaatggcaacaacgttgcgcaaactattaactggcgaactacttactctagcttcccggcaacaattaatagactggatggaggcggataaagttgcaggaccacttctgcgctcggcccttccggctggctggtttattgctgataaatctggagccggtgagcgtgggtctcgcggtatcattgcagcactggggccagatggtaagccctcccgtatcgtagttatctacacgacggggagtcaggcaactatggatgaacgaaatagacagatcgctgagataggtgcctcactgattaagcattggtaactgtcagaccaagtttactcatatatactttagattgatttaaaacttcatttttaatttaaaaggatctaggtgaagatcctttttgataatctcatgaccaaaatcccttaacgtgagttttcgttccactgagcgtcagaccccgtagaaaagatcaaaggatcttcttgagatcctttttttctgcgcgtaatctgctgcttgcaaacaaaaaaaccaccgctaccagcggtggtttgtttgccggatcaagagctaccaactctttttccgaaggtaactggcttcagcagagcgcagataccaaatactgtccttctagtgtagccgtagttaggccaccacttcaagaactctgtagcaccgcctacatacctcgctctgctaatcctgttaccagtggctgctgccagtggcgataagtcgtgtcttaccgggttggactcaagacgatagttaccggataaggcgcagcggtcgggctgaacggggggttcgtgcacacagcccagcttggagcgaacgacctacaccgaactgagatacctacagcgtgagctatgagaaagcgccacgcttcccgaagggagaaaggcggacaggtatccggtaagcggcagggtcggaacaggagagcgcacgagggagcttccagggggaaacgcctggtatctttatagtcctgtcgggtttcgccacctctgacttgagcgtcgatttttgtgatgctcgtcaggggggcggagcctatggaaaaacgccagcaacgcggcctttttacggttcctggccttttgctggccttttgctcacatgttctttcctgcgttatcccctgattctgtggataaccgtattaccgcctttgagtgagctgataccgctcgccgcagccgaacgaccgagcgcagcgagtcagtgagcgaggaagcggaagagcgcccaatacgcaaaccgcctctccccgcgcgttggccgattcattaatgcagggggatctcgatcccgcgaaattaatacgactcactatagtctcaaagacatcaatccccccgttacccacgttaacacagagagctctagtagtggtctttccttttgtgaaaccatggacttcttgagaagccttgactggactcaagtgattgctggtcaatatgtgtccaaccctaggttcaacatttctgattattttgagattgtgcggcagcctggtgatgggaactgcttctatcacagcatagctgagttaaccatgcctaacaaaacagatcactcatatcattacatcaaacgcctaaccgagtcggcagcacggaagtattaccaagaggagcctgaagccagacttgttggcctgagcctggaagattacctcaagaggatgctgtctgacaacgagtggggatcaactctagaagcatctatgttggctaaagaaatgggcattaccatcatcatttggactgttgctgccagtgatgaagtggaagcaggtataaagttcggagacggtgatgtgtttacagctgtgaaccttttgcactctggacaaacacactttgatgcgctcagaatacttccgcagtttgaaacagacacaagagaggccttgagcttgatggacagggttatagctgtggatcagttgacatcatcttctagtgatgaactgcaagactatgaagaccttgccttggcactcacaagcgcagaagaatcaaatagacggtcaagcttggatgaggtcacattgtccaagaagcaagcagagatactaaggcaaaaagcatctcagttgtctaaattggttaataaaagtcagaacataccgaccagagtcggtagagtcttggattgcatgttcaactgcaaattatgtgttgagatatcagctgacactttaattctgaggccagaatcaaaagagaaaatcggtgaaatcatgtcattgcggcagttggggcataaactgctgacacgagacaaacagattaagcaagagttctccagaatgaaactctacgtcactaaagatttgcttgaccatctagacgttggtgggctcttgagggctgctttccctggaacaggaatagaaaggcatatgcagctgctacactctgagatgatactggacatctgcactgtatcacttggtgtcatgctgtcaacattcttatatggttctaataataaaaacaagaagaaattcattaccaactgtctgctcagcacagccctatccggaaagaaggtgtataaagttctcggcaacctaggaaatgaactgttgtacaaggcacctagaaaggccttagcaactgtctgcagtgccttgtttgggaagcagataaacaaacttcagaattgcttcaggaccataagccctgtcagcttacttgcattgagaaatctagactttgattgtctcagtgtgcaagactataatggtatgatagaaaacatgtctaaattagacaacactgatgttgaattcaaccacagggagatagctgatctcaaccaattaacttctcggctcatcacattaagaaaggagaaagacactgacctcctcaaacaatggtttcctgaaagtgacctcacccgcagaagcatcaggaatgctgcaaacgcggaggaatttgtcatatctgagttctttaagaagaaggacattatgaaattcatcagcacttcaggcagagcaatgagtgcaggcaagattggtaatgtcctatcctatgcacataatctttatttgagtaagtcaagcctaaatatgacctctgaagacatctcacagcttttgatcgagattaagcgactgtatgctttacaagaagattctgaagtggagccgatagccataatttgtgatggcatagaaagcaacatgaaacagttatttgctatattgcctcctgactgtgcaagagagtgtgaagtcctcttcgatgacataagaaattctccaacacacagcacagcctggaagcatgcactccgattaaaagggactgcatacgaaggtctgtttgcaaattgttacggctggcaatacattccggaagacattaaaccaagcctgaccatgttgatacagactttgtttcctgacaagttcgaagatttcctggatcgaacccagttgcatccggagttcagagacctgactcccgacttttcgctcacacaaaaggttcactttaaaagaaatcagatacccagtgtcgaaaatgtgcaaatctccattgatgcgacgttgcctgaatctgtggaagcagtaccagtgacagaaagaaagatgttcccccttcctgagactccgctaagtgaggtgcattcaatagagcgtataatggaaaactttactcgcctcatgcatggaggaagactttcgaccaagaaaagagatggagatccggcggaacagggcaaccagcagagtatcactgaacacgagagttccagcatctctgcctttaaagactacggagagagagggatagtcgaggaaaatcacatgaagtttagtggagaagatcagctagagacaaggcagctgttgttggtggaagttggttttcaaactgacatcgatgggaaaataaggacagaccacaagaagtggaaagacatattaaagctattagagctactaggaatcaagtgctcattcattgcctgtgcagattgctcatccacaccaccagacagatggtggattacggaggacagagtgcgagtcctaaaaaattcagtcagcttcttgttcaataaactctccagaaactcacctacagaagtaactgacatagttgttggagctataagtactcaaaaggttagaagttatctaaaggcaggaactgcaacaaaaacccctgtgtcgactaaagacgttctggagacttgggaaaagatgaaggagcacatactcaacagaccaacaggactgacactgcccaccagtttggaacaggcaatgcgcaaaggactggtcgaaggtgtggtcatctccaaggaaggttctgagtcatgtatcaatatgttgaaggaaaatttggaccgaataactgacgaattcgagcgaacaaaatttaaacatgaacttactcagaatattaccacaagtgagaagatgctattgagttggttgagtgaagacatcaaatcatcgagatgtggtgagtgcctctcaaatataaagaaagccgttgatgaaactgccaatctatcagaaaagattgagctgctcgcttataatctgcaactcaccaatcactgcagcaactgtcaccccaatggtgtaaacattagtaacacttctaatgtgtgcaagagatgccccaagattgaagtggttagccattgtgaaaataaaggctttgaggacagcaatgaatgcttaacagacctagataggcttgttaggctcacattaccagggaaaactgagaaggagagaagagtcaaacgtaatgtggaatatcttataaaactgatgatgagcatgtcaggcattgattgtataaaatatcccacagggcagcttatcacccatggaagagtgagtgcaaaacataacgatgggaacctgaaagatagaagcgatgacgaccaaagactagctgagaagatagacactgttaggaaagagctttcagaatctaaactgaaagattattcaacttatgcaaggggagtgatatcaaattcactaaaaaacctctcaaggcaaggtaaatcaaagtgttctgtgccaagatcttggctcgagaaagtactgtttgacctgaaggtgcctactaaggacgaagaagtgcttataaacatcagaaactcattgaaagctagatccgagtttgttagaaataacgataaactactcataaggtcaaaagaagaactaaaaaaatgtttcgatgtgcagtcttttaaattgaaaaaaaacaagcaacctgtgccctttcaggttgactgtatattgttcaaagaagtggcagctgaatgcatgaagaggtacattggcacaccttatgagggaattgtagacaccttagtttctctgattaatgtgttaacaaggtttacttggttccaggaagtggtgctatatggtaaaatatgtgagaccttcctaagatgctgcacagaatttaataggtcaggggtcaaactggttaagataaggcactgtaacattaacctatcagtcaaattgccatcaaataagaaagagaatatgttatgttgtctatatagtggaaacatggagctcttgcaaggacctttctatttgaacaggagacaagctgtccttggttcttcatacctttacattgtcattacactttacatacaagtgctgcagcagtacaggtgtctagaagttataaacagtgtgagtgaaaaaacattgcaagacattgaaaatcattccatgactctactagaagattcattcagggaaatcacttttgctcttgaaggtaggtttgaagaatcttataaaatacgaacctcgaggtgcagagccagtgggaattttctgaacaggagcagtagagaccactttataagcgttgtttcaggcttgaacctagtttatggcttcctcataaaagataacttactagccaactctcagcaacagaacaaacaactacagatgcttcgttttggcatgcttgcagggcttagtaggcttgtttgtcctaatgagctaggaaagaaattttcaacgagctgtagaagaattgaagacaacattgcaaggctttacctgcagacatccatttactgttcagtcagggatgtggaggacaatgttaagcactggaaacaaagagatctatgtcctgaagtaaccattccatgctttacagtctatggaacctttgtcaacagcgatagacaactgatctttgacatttacaatgtgcatatatataataaagaaatggacaactttgatgaaggatgtatcagcgtcttggaagaaacagcagaaaggcacatgctttgggaactcgatctgatgaattcactttgttctgacgaaaaaaaagatactagaaccgcaagactattactaggctgcccaaatgtgaggaaagcagcaaacagagaagggaagaagctgttgaagttaaacagtgacacatccacagacacacagagcattgcttctgaagtgtcggacagaaggtcttatagttcaagtaagagtagaatccgtagtatatttggtagatacaactctcagaagaaaccatttgaattaaggtcaggtcttgaggttttcaatgatcctttcaatgattatcagcaagcaataacggacatttgccaattttctgagtacacaccaaacaaagaaagcattttgaaagactgtcttcaaatcatacgaaaaaaccctagccacacaatgggttcttttgagctgatccaggcaatctcagagttcggcatgagcaagtttcctcccgaaaatatagacaaagcaagaagggatccgaagaactgggttagcatctctgaagtaaccgaaacaacaagtatagttgcatcacctagaactcatatgatgctcaaggattgttttaaaattatactaggtactgagaataagaagatagtcaaaatgcttcgaggtaagctaaagaaactcggtgctatctcaacaaacatagagatcgggaaaagggattgcctagatctactcagcacagtagatgggctaacagaccagcagaaagaaaatattgtaaatgggatatttgagccctcaaagttatccttctaccattggaaggaattggtcaaaaaaaacattgatgaagttttacttactgaagatggaaatctgatcttctgctggctgaaaacaatctcctcttcagtcaaaggaagcctaaagaagagactcaaattcatgaatatacattctccagaattgatgccggaaaactgtctcttttctagtgaggaattcaatgagttaattaagttgaagaaactcctcctcaatgaacaacaagatgaacaggagctgaaacaagatcttttgatatcttcttggatcaagtgcataacagcttgcaaggattttgcaagcatcaatgacaagattcagaagttcatttaccacctgtctgaagagctatatgacataaggctgcagcatctggaactgtcaaagcttaagcaagagcaccctagtgtcagcttcacaaaagaagaagtcttaataaagcggctggagaaaaatttccttaagcagcataatttagagattatggaaactgtgaatcttgtattctttgcagccctctcagctccctggtgcttacactataaagcactagagtcttatttggtgagacatccagaaatacttgactgtggatctaaggaggactgcaaactcaccttgcttgatctgtcagtttctaagctcttggtttgtttgtatcaaaaagatgatgaggagctgataaatagctcaagtttgaaacttgggtttttagtgaaatatgttgtcaccttgttcacatccaatggtgaacctttttcactcagtctcaatgacgggggtttggatcttgatttacacaagactactgacgaaaagttactacatcaaacaaagatagtttttgctaaaattggtttatctgggaacagttatgactttatctggactacccaaatgatagcaaacagcaattttaacgtctgcaaaagattaacgggaaggagtactggggaaaggctccctagaagcgttagaagcaaggtcatatatgagatggtaaaattagtgggagaaacaggcatggcaatactacaacaattagcttttgcacaagcactaaattatgagcaccgcttctatgcggtcttagcacctaaagcgcaactaggaggagcaagagatttgttagtgcaagagactgggactaaagtcatgcatgcaaccactgaaatgtttagtagaaatcttttaaaaacaacatcagatgatggcctcacaaacccacatcttaaagaaacaatccttaatgtgggattagactgtcttgctaacatgcgaaatcttgacggtaagcccataagtgaaggtagtaacttggtcaatttctacaaagtcatatgtatctcgggtgataataccaagtggggcccgatacactgctgttctttcttttctggcatgatgcaacaggttctgaaaaatgtaccagattggtgttcattttataaattaacattcattaaaaacttatgtagacaggtagaaatacctgctggcagtattaagaagatcttaaatgttcttaggtatagattgtgcagcaagggaggtgtagaacaacatagtgaagaagatctgagaagactgttgacagataatttagacagttgggatggaaacgacacagttaagttcttagttacaacttatataagcaaaggactcatggcgttaaacagttacaatcatatgggtcagggtattcaccatgcaacatcttcggtgttaacttccctagctgctgtgctctttgaggagctggcaattttttatcttaagagaagcttaccccagacaacagtacatgttgaacatgccggtagttcagatgattacgcaaagtgtatagtggtgactggtatactatccaaagagctctactcccagtatgatgaaacattttggaaacacgcttgcagactcaaaaacttcacggccgcggtacaaagatgctgtcaaatgaaagatagtgccaaaaccttggtgagcgactgctttctcgagttttacagtgagtttatgatgggctacagagtaacccctgctgtaataaagttcatgtttactggactgataaacagctctgtgacctctcctcagagtttgatgcaagcatgccaagtttcatcccaacaagcaatgtataatagtgttcctcttgtcaccaacactgccttcaccctattaaggcagcaaattttctttaaccatgttgaagactttatcagaaggtatggtatactgactcttgggactttgtcaccctttggtaggttgttcgtaccaacctactctggattagtcagctcagcggttgctttagaagatgctgaagtcattgctagagcagcccaaacacttcaaatgaacagtgtgtcaatacagtcaagtagcttgaccacattagatagcctaggtcgtagtaggacaagttccacagctgaggatagcagcagtgtgagcgacacaactgctgcttcccatgactcaggatcatcatcctcaagcttctcttttgagctcaatagacccctgtctgaaactgaactacagttcattaaagcactaagtagtctcaagtcaacacaagcctgtgaagtgattcaaaatagaattacaggtctttattgcaacagcaacgaaggacctcttgataggcataatgtcatttacagcagcagaatggcagactcttgcgattggctaaaggatggtaaaaggagagggaatctagaactagcgaataggatccaatctgtactgtgtattctgatagcaggatattacaggtcatttggaggggaaggaaccgagaaacaggtaaaggcatcattgaatagagacgacaataaaatcatagaggatcctatgatacaactaattccagaaaagctgaggagagagttagaaaggttaggtgtttctagaatggaagtcgatgagctaatgccaagcattagtcctgatgacaccttagcccagcttgtagcgaaaaaactcattagcctcaatgtttcgacagaagaatactcagctgaggtatctagactcaaacaaacactgacagcccgaaatgttttgcacgggttagctggagggattaaggagctttcgcttccaatatatacaatattcatgaaatcttacttctttaaagacaatgttttcctgtcactaacagatagatggtctaccaagcacagtacaaactatcgtgatagttgtggcaaacaattaaaaggtagaataattaccaagtatactcactggttggacacttttctgggctgctctgtctccatcaacaggcatactactgttaaagagccctccttattcaatccgaacatcagatgtgtgaatctgatcacatttgaggacggcctgagagaactatcagtgatacagagtcaccttaaagtctttgaaaatgagttcaccaacttaaatcttcaattctctgatccgaacagacagaaacttagaatagttgagtctagacctgcagaatctgagctagaggcaaaccgtgcagtaattgtcaagaccaaattgttttcagcaactgaacaagttcgactatccaacaaccctgcagttgtcatgggctacctattggatgaatcagcaatttcagaagtcaagcctaccaaggttgacttctcaaatttacttaaagaccgcttcaaaataatgcaattttttccttcagtgttcactttgattaagatgctgacagatgaatcgtcagattcagaaaagagtggccttagtccagatttgcaacaagttgcaagatactcaaaccatttgaccttgctcagcagaatgattcaacaagcaaagccaaccgtgactgttttctacatgctaaaaggtaacttgatgaacacagagccaacagttgctgagcttgtcagctatggtataaaggaaggcagattttttaggctttccgacaccggagtcgatgcaagcacatactctgtaaaatattggaaaattcttcactgcatctctgccattggatgtttacctttgagtcaagcagacaaatcttcactacttatgagcttcttaaactggagggtcaacatggacattagaacatctgactgtccactatctagtcatgaagcaagtatactgagtgaatttgatggacaagttatcgccaacatacttgccagtgaattgagttctgtgaaacgagattctgaacgcgagggtctaactgatctccttgattatctaaactcaccaactgaattgttgaagaagaagccttacttagggacaacttgcaagttcaacacctggggagactcgaatagatctggaaagttcacatacagcagcagatctggagaatccattggaatcttcattgcagggaaattgcacatccatctctcatctgagtccgttgccttgttgtgtgaaactgaaagacaagtgctttcttggatgagtaagaggaggactgaggtaataactaaagaacagcatcaactgtttctaagtcttctcccacagtctcatgagtgtttacaaaagcacaaggacggtagtgcgctatcagtcatacctgatagcagcaacccccgattacttaagtttgtgcccctcaaaaaaggtctagcagtggtgaaaatcaaaaaacaaattttaacagtgaagaagcaggttgtgtttgatgcagagagcgagcctagactgcagtgggggcatggctgcttgtccattgtttatgacgaaactgatactcagaccacataccatgaaaatcttttgaaggtgaagcatcttgtagactgctctacagatagaaaaaagcttttgccccagtcagtgttttctgactccaaagttgtcctttcaaggatcaagttcaagacggagcttctcctcaactcattgacgctgctccactgtttcctaaaacatgctcctagtgatgccataatggaggtagagagcaaaagtagcttgctacacaagtacctcaaatcgggaggtgtcaggcaacggaacactgaagtgctcttcagagagaagttaaacaaggttgttataaaagacaatcttgagcaaggtgtggaagaggagattgagttttgcaacaacttgactaagactgtttcagagaacccattaccactcagctgttggtctgaagttcaaaattacattgaagacataggctttaacaatgtacttgttaacattgacagaaacacggtgaaaagtgaacttttatggaaatttacgttagacaccaatgtaagcaccacaagtactataaaagacgtgaggacattggtgtcctacgttagcactgaaaccatccctaagttcttgcttgcattcttactttatgaagaagtgttaatgaacttaatcaaccagtgtaaggcagtaaaagaactcatcaacagcacaggactctcagacttggaactggaaagcttactcactttatgtgctttctatttccaaagtgagtgcagtaagagagatggtcctagatgctcctttgcagcactattaagtctaatccatgaggattggcagaggataggtaaaaacattcttgttcgtgcaaacaatgaactaggtgatgtgtcactgaaggttaacattgtcctggtgcctctcaaggacatgtctaagccaaagtctgagagagtggtcatggctagaaggtcactaaatcatgctctatccttgatgtttctggacgagatgtcactacctgagctaaaatccttatccgtgaactgcaaaatggggaactttgaagggcaggagtgctttgagttcactattctgaaggacaatagcgcaagactagattacaacaagttgattgaccactgtgtggacatggaaaaaaagagggaagcggttagagcagtagaagatttaattttgatgttgacaggcagagcagtcaaacccagcgctgtaacacagtttgtacacggggacgagcagtgtcaagagcaaataagcttagatgatctgatggcaaacgacacggtaacagactttcctgatagggaagcagaagccctcaaaacaggaaatcttggctttaactgggactcagattgaacatgccgcttataagccattaatacctttcggcgtcacaaggacaaatgatgcagttttagctgcatcattcattaacattaaagccttcaaacaagctaactactctgcattctcctcaatcaactcaattgcttcaactgatctattttactagctcatcgatcctctctttcttagctattcatttcagcttcatcatcatcgttattatcttggggtgtggggggaacgatttctttgagagggtcggcatggcatctccacctcctcgcggtccgacctgggcatccgaaggaggacgtcgtccactcggatggctaagggagagctcggatccggctgctaacaaagcccgaaaggaagctgagttggctgctgccaccgctgagcaataactagcataaccccttggggcctctaaacgggtcttgaggggtttttt

SEQ ID NO: 3 - DNA, 6225 bp, Artificial Sequence
  Synthetic construct (pC-N)
gtcgacattgattattgactagttattaatagtaatcaattacggggtcattagttcatagcccatatatggagttccgcgttacataacttacggtaaatggcccgcctggctgaccgcccaacgacccccgcccattgacgtcaataatgacgtatgttcccatagtaacgccaatagggactttccattgacgtcaatgggtggactatttacggtaaactgcccacttggcagtacatcaagtgtatcatatgccaagtacgccccctattgacgtcaatgacggtaaatggcccgcctggcattatgcccagtacatgaccttatgggactttcctacttggcagtacatctacgtattagtcatcgctattaccatgggtcgaggtgagccccacgttctgcttcactctccccatctcccccccctccccacccccaattttgtatttatttattttttaattattttgtgcagcgatgggggcggggggggggggggcgcgcgccaggcggggcggggcggggcgaggggcggggcggggcgaggcggagaggtgcggcggcagccaatcagagcggcgcgctccgaaagtttccttttatggcgaggcggcggcggcggcggccctataaaaagcgaagcgcgcggcgggcgggagtcgctgcgttgccttcgccccgtgccccgctccgcgccgcctcgcgccgcccgccccggctctgactgaccgcgttactcccacaggtgagcgggcgggacggcccttctcctccgggctgtaattagcgcttggtttaatgacggctcgtttcttttctgtggctgcgtgaaagccttaaagggctccgggagggccctttgtgcgggggggagcggctcggggggtgcgtgcgtgtgtgtgtgcgtggggagcgccgcgtgcggcccgcgctgcccggcggctgtgagcgctgcgggcgcggcgcggggctttgtgcgctccgcgtgtgcgcgaggggagcgcggccgggggcggtgccccgcggtgcgggggggctgcgaggggaacaaaggctgcgtgcggggtgtgtgcgtgggggggtgagcagggggtgtgggcgcggcggtcgggctgtaacccccccctgcacccccctccccgagttgctgagcacggcccggcttcgggtgcggggctccgtgcggggcgtggcgcggggctcgccgtgccgggcggggggtggcggcaggtgggggtgccgggcggggcggggccgcctcgggccggggagggctcgggggaggggcgcggcggccccggagcgccggcggctgtcgaggcgcggcgagccgcagccattgccttttatggtaatcgtgcgagagggcgcagggacttcctttgtcccaaatctggcggagccgaaatctgggaggcgccgccgcaccccctctagcgggcgcgggcgaagcggtgcggcgccggcaggaaggaaatgggcggggagggccttcgtgcgtcgccgcgccgccgtccccttctccatctccagcctcggggctgccgcagggggacggctgccttcgggggggacggggcagggcggggttcggcttctggcgtgtgaccggcggctctagagcctctgctaaccatgttcatgccttcttctttttcctacagctcctgggcaacgtgctggttgttgtgctgtctcatcattttggcaaagaattcgagctcatcgatgcatggttctcttgatggaaaacaagatcgaggtgaataacaaagatgagatgaacaggtggtttgaagagttcaaaaaaggaaatggacttgtggacaccttcacaaactcctattccttttgcgagagtgttcccaatttggacaggtttgtgtttcagatggccagtgccaccgatgatgcacagaaggactccatctacgcatctgctctggtggaggcaacaaagttttgtgcacctatatatgagtgcgcatgggttagctccactggcattgtaaaaaagggacttgaatggttcgagaaaaatgcaggaaccattaagtcctgggatgaaagttatactgagctaaaggtcgacgtcccgaaaatagagcagcttaccggttaccaacaagctgccttgaagtggagaaaagacataggtttccgtgtcaatgccaacacagcagctctgagcaacaaagtcctcgcagaatacaaagtccctggtgagattgtgatgtctgtcaaagagatgctgtcagacatgattaggagaaggaacctgattctaaacaggggtggtgatgagaacccacgtggcccagtgagccatgagcatgtagactggtgcagggagtttgtcaaaggcaaatacatcatggccttcaacccaccatggggggacatcaacaagtcaggccgttcaggaatagcacttgttgcaacaggccttgctaagcttgcagagactgaaggaaagggaatatttgatgaagccaaaaagactgtggaggccctcaacgggtatctggacaagcataaggacgaagttgatagagcaagcgccgacagcatgataacaaaccttcttaagcatattgccaaggcacaggagctctataaaaattcatctgcacttcgtgcacaaagcgcacagattgacactgctttcagctcatactattggctttacaaggctggcgtgactcctgaaaccttcccgacggtgtcacagttcctctttgagctagggaaacagccaagaggtaccaagaaaatgaagaaggctcttctgagcaccccaatgaagtgggggaagaagctttatgagctctttgccgatgattctttccagcagaacaggatttacatgcatcctgccgtgcttacagctggtagaatcagtgaaatgggagtctgctttgggacaatccctgtggccaatcctgatgatgctgcccaaggatctggacacactaagtctattctcaacctccgtaccaacactgagaccaataatccgtgtgccaaaaccatcgtcaagctatttgaagttcaaaaaacagggttcaacattcaggacatggacatagtggcctctgagcacttgctacaccaatcccttgttggcaagcaatccccattccagaacgcctacaacgtcaagggcaatgccaccagtgctaacatcatttaaaatacaaactgctctgtactcaacttccgggcatgctcgagctagcagatctttttccctctgccaaaaattatggggacatcatgaagccccttgagcatctgacttctggctaataaaggaaatttattttcattgcaatagtgtgttggaattttttgtgtctctcactcggaaggacatatgggagggcaaatcatttaaaacatcagaatgagtatttggtttagagtttggcaacatatgccatatgctggctgccatgaacaaaggtggctataaagaggtcatcagtatatgaaacagccccctgctgtccattccttattccatagaaaagccttgacttgaggttagattttttttatattttgttttgtgttatttttttctttaacatccctaaaattttccttacatgttttactagccagatttttcctcctctcctgactactcccagtcatagctgtccctcttctcttatgaagatccctcgacctgcagcccaagcttggcgtaatcatggtcatagctgtttcctgtgtgaaattgttatccgctcacaattccacacaacatacgagccggaagcataaagtgtaaagcctggggtgcctaatgagtgagctaactcacattaattgcgttgcgctcactgcccgctttccagtcgggaaacctgtcgtgccagcggatccgcatctcaattagtcagcaaccatagtcccgcccctaactccgcccatcccgcccctaactccgcccagttccgcccattctccgccccatggctgactaattttttttatttatgcagaggccgaggccgcctcggcctctgagctattccagaagtagtgaggaggcttttttggaggcctaggcttttgcaaaaagctaacttgtttattgcagcttataatggttacaaataaagcaatagcatcacaaatttcacaaataaagcatttttttcactgcattctagttgtggtttgtccaaactcatcaatgtatcttatcatgtctggatccgctgcattaatgaatcggccaacgcgcggggagaggcggtttgcgtattgggcgctcttccgcttcctcgctcactgactcgctgcgctcggtcgttcggctgcggcgagcggtatcagctcactcaaaggcggtaatacggttatccacagaatcaggggataacgcaggaaagaacatgtgagcaaaaggccagcaaaaggccaggaaccgtaaaaaggccgcgttgctggcgtttttccataggctccgcccccctgacgagcatcacaaaaatcgacgctcaagtcagaggtggcgaaacccgacaggactataaagataccaggcgtttccccctggaagctccctcgtgcgctctcctgttccgaccctgccgcttaccggatacctgtccgcctttctcccttcgggaagcgtggcgctttctcaatgctcacgctgtaggtatctcagttcggtgtaggtcgttcgctccaagctgggctgtgtgcacgaaccccccgttcagcccgaccgctgcgccttatccggtaactatcgtcttgagtccaacccggtaagacacgacttatcgccactggcagcagccactggtaacaggattagcagagcgaggtatgtaggcggtgctacagagttcttgaagtggtggcctaactacggctacactagaaggacagtatttggtatctgcgctctgctgaagccagttaccttcggaaaaagagttggtagctcttgatccggcaaacaaaccaccgctggtagcggtggtttttttgtttgcaagcagcagattacgcgcagaaaaaaaggatctcaagaagatcctttgatcttttctacggggtctgacgctcagtggaacgaaaactcacgttaagggattttggtcatgagattatcaaaaaggatcttcacctagatccttttaaattaaaaatgaagttttaaatcaatctaaagtatatatgagtaaacttggtctgacagttaccaatgcttaatcagtgaggcacctatctcagcgatctgtctatttcgttcatccatagttgcctgactccccgtcgtgtagataactacgatacgggagggcttaccatctggccccagtgctgcaatgataccgcgagacccacgctcaccggctccagatttatcagcaataaaccagccagccggaagggccgagcgcagaagtggtcctgcaactttatccgcctccatccagtctattaattgttgccgggaagctagagtaagtagttcgccagttaatagtttgcgcaacgttgttgccattgctacaggcatcgtggtgtcacgctcgtcgtttggtatggcttcattcagctccggttcccaacgatcaaggcgagttacatgatcccccatgttgtgcaaaaaagcggttagctccttcggtcctccgatcgttgtcagaagtaagttggccgcagtgttatcactcatggttatggcagcactgcataattctcttactgtcatgccatccgtaagatgcttttctgtgactggtgagtactcaaccaagtcattctgagaatagtgtatgcggcgaccgagttgctcttgcccggcgtcaatacgggataataccgcgccacatagcagaactttaaaagtgctcatcattggaaaacgttcttcggggcgaaaactctcaaggatcttaccgctgttgagatccagttcgatgtaacccactcgtgcacccaactgatcttcagcatcttttactttcaccagcgtttctgggtgagcaaaaacaggaaggcaaaatgccgcaaaaaagggaataagggcgacacggaaatgttgaatactcatactcttcctttttcaatattattgaagcatttatcagggttattgtctcatgagcggatacatatttgaatgtatttagaaaaataaacaaataggggttccgcgcacatttccccgaaaagtgccacctg

SEQ ID NO: 4 - DNA, 16635 bp, Artificial Sequence
  Synthetic construct (pC-L)
gtcgacattgattattgactagttattaatagtaatcaattacggggtcattagttcatagcccatatatggagttccgcgttacataacttacggtaaatggcccgcctggctgaccgcccaacgacccccgcccattgacgtcaataatgacgtatgttcccatagtaacgccaatagggactttccattgacgtcaatgggtggactatttacggtaaactgcccacttggcagtacatcaagtgtatcatatgccaagtacgccccctattgacgtcaatgacggtaaatggcccgcctggcattatgcccagtacatgaccttatgggactttcctacttggcagtacatctacgtattagtcatcgctattaccatgggtcgaggtgagccccacgttctgcttcactctccccatctcccccccctccccacccccaattttgtatttatttattttttaattattttgtgcagcgatgggggcggggggggggggggcgcgcgccaggcggggcggggcggggcgaggggcggggcggggcgaggcggagaggtgcggcggcagccaatcagagcggcgcgctccgaaagtttccttttatggcgaggcggcggcggcggcggccctataaaaagcgaagcgcgcggcgggcgggagtcgctgcgttgccttcgccccgtgccccgctccgcgccgcctcgcgccgcccgccccggctctgactgaccgcgttactcccacaggtgagcgggcgggacggcccttctcctccgggctgtaattagcgcttggtttaatgacggctcgtttcttttctgtggctgcgtgaaagccttaaagggctccgggagggccctttgtgcgggggggagcggctcggggggtgcgtgcgtgtgtgtgtgcgtggggagcgccgcgtgcggcccgcgctgcccggcggctgtgagcgctgcgggcgcggcgcggggctttgtgcgctccgcgtgtgcgcgaggggagcgcggccgggggcggtgccccgcggtgcgggggggctgcgaggggaacaaaggctgcgtgcggggtgtgtgcgtgggggggtgagcagggggtgtgggcgcggcggtcgggctgtaacccccccctgcacccccctccccgagttgctgagcacggcccggcttcgggtgcggggctccgtgcggggcgtggcgcggggctcgccgtgccgggcggggggtggcggcaggtgggggtgccgggcggggcggggccgcctcgggccggggagggctcgggggaggggcgcggcggccccggagcgccggcggctgtcgaggcgcggcgagccgcagccattgccttttatggtaatcgtgcgagagggcgcagggacttcctttgtcccaaatctggcggagccgaaatctgggaggcgccgccgcaccccctctagcgggcgcgggcgaagcggtgcggcgccggcaggaaggaaatgggcggggagggccttcgtgcgtcgccgcgccgccgtccccttctccatctccagcctcggggctgccgcagggggacggctgccttcgggggggacggggcagggcggggttcggcttctggcgtgtgaccggcggctctagagcctctgctaaccatgttcatgccttcttctttttcctacagctcctgggcaacgtgctggttgttgtgctgtctcatcattttggcaaagaattcgagctcatcgatgcatgaccggtaaccatgggtaagcctatccctaaccctctcctcggtctcgattctacgatggacttcttgagaagccttgactggactcaagtgattgctggtcaatatgtgtccaaccctaggttcaacatttctgattattttgagattgtgcggcagcctggtgatgggaactgcttctatcacagcatagctgagttaaccatgcctaacaaaacagatcactcatatcattacatcaaacgcctaaccgagtcggcagcacggaagtattaccaagaggagcctgaagccagacttgttggcctgagcctggaagattacctcaagaggatgctgtctgacaacgagtggggatcaactctagaagcatctatgttggctaaagaaatgggcattaccatcatcatttggactgttgctgccagtgatgaagtggaagcaggtataaagttcggagacggtgatgtgtttacagctgtgaaccttttgcactctggacaaacacactttgatgcgctcagaatacttccgcagtttgaaacagacacaagagaggccttgagcttgatggacagggttatagctgtggatcagttgacatcatcttctagtgatgaactgcaagactatgaagaccttgccttggcactcacaagcgcagaagaatcaaatagacggtcaagcttggatgaggtcacattgtccaagaagcaagcagagatactaaggcaaaaagcatctcagttgtctaaattggttaataaaagtcagaacataccgaccagagtcggtagagtcttggattgcatgttcaactgcaaattatgtgttgagatatcagctgacactttaattctgaggccagaatcaaaagagaaaatcggtgaaatcatgtcattgcggcagttggggcataaactgctgacacgagacaaacagattaagcaagagttctccagaatgaaactctacgtcactaaagatttgcttgaccatctagacgttggtgggctcttgagggctgctttccctggaacaggaatagaaaggcatatgcagctgctacactctgagatgatactggacatctgcactgtatcacttggtgtcatgctgtcaacattcttatatggttctaataataaaaacaagaagaaattcattaccaactgtctgctcagcacagccctatccggaaagaaggtgtataaagttctcggcaacctaggaaatgaactgttgtacaaggcacctagaaaggccttagcaactgtctgcagtgccttgtttgggaagcagataaacaaacttcagaattgcttcaggaccataagccctgtcagcttacttgcattgagaaatctagactttgattgtctcagtgtgcaagactataatggtatgatagaaaacatgtctaaattagacaacactgatgttgaattcaaccacagggagatagctgatctcaaccaattaacttctcggctcatcacattaagaaaggagaaagacactgacctcctcaaacaatggtttcctgaaagtgacctcacccgcagaagcatcaggaatgctgcaaacgcggaggaatttgtcatatctgagttctttaagaagaaggacattatgaaattcatcagcacttcaggcagagcaatgagtgcaggcaagattggtaatgtcctatcctatgcacataatctttatttgagtaagtcaagcctaaatatgacctctgaagacatctcacagcttttgatcgagattaagcgactgtatgctttacaagaagattctgaagtggagccgatagccataatttgtgatggcatagaaagcaacatgaaacagttatttgctatattgcctcctgactgtgcaagagagtgtgaagtcctcttcgatgacataagaaattctccaacacacagcacagcctggaagcatgcactccgattaaaagggactgcatacgaaggtctgtttgcaaattgttacggctggcaatacattccggaagacattaaaccaagcctgaccatgttgatacagactttgtttcctgacaagttcgaagatttcctggatcgaacccagttgcatccggagttcagagacctgactcccgacttttcgctcacacaaaaggttcactttaaaagaaatcagatacccagtgtcgaaaatgtgcaaatctccattgatgcgacgttgcctgaatctgtggaagcagtaccagtgacagaaagaaagatgttcccccttcctgagactccgctaagtgaggtgcattcaatagagcgtataatggaaaactttactcgcctcatgcatggaggaagactttcgaccaagaaaagagatggagatccggcggaacagggcaaccagcagagtatcactgaacacgagagttccagcatctctgcctttaaagactacggagagagagggatagtcgaggaaaatcacatgaagtttagtggagaagatcagctagagacaaggcagctgttgttggtggaagttggttttcaaactgacatcgatgggaaaataaggacagaccacaagaagtggaaagacatattaaagctattagagctactaggaatcaagtgctcattcattgcctgtgcagattgctcatccacaccaccagacagatggtggattacggaggacagagtgcgagtcctaaaaaattcagtcagcttcttgttcaataaactctccagaaactcacctacagaagtaactgacatagttgttggagctataagtactcaaaaggttagaagttatctaaaggcaggaactgcaacaaaaacccctgtgtcgactaaagacgttctggagacttgggaaaagatgaaggagcacatactcaacagaccaacaggactgacactgcccaccagtttggaacaggcaatgcgcaaaggactggtcgaaggtgtggtcatctccaaggaaggttctgagtcatgtatcaatatgttgaaggaaaatttggaccgaataactgacgaattcgagcgaacaaaatttaaacatgaacttactcagaatattaccacaagtgagaagatgctattgagttggttgagtgaagacatcaaatcatcgagatgtggtgagtgcctctcaaatataaagaaagccgttgatgaaactgccaatctatcagaaaagattgagctgctcgcttataatctgcaactcaccaatcactgcagcaactgtcaccccaatggtgtaaacattagtaacacttctaatgtgtgcaagagatgccccaagattgaagtggttagccattgtgaaaataaaggctttgaggacagcaatgaatgcttaacagacctagataggcttgttaggctcacattaccagggaaaactgagaaggagagaagagtcaaacgtaatgtggaatatcttataaaactgatgatgagcatgtcaggcattgattgtataaaatatcccacagggcagcttatcacccatggaagagtgagtgcaaaacataacgatgggaacctgaaagatagaagcgatgacgaccaaagactagctgagaagatagacactgttaggaaagagctttcagaatctaaactgaaagattattcaacttatgcaaggggagtgatatcaaattcactaaaaaacctctcaaggcaaggtaaatcaaagtgttctgtgccaagatcttggctcgagaaagtactgtttgacctgaaggtgcctactaaggacgaagaagtgcttataaacatcagaaactcattgaaagctagatccgagtttgttagaaataacgataaactactcataaggtcaaaagaagaactaaaaaaatgtttcgatgtgcagtcttttaaattgaaaaaaaacaagcaacctgtgccctttcaggttgactgtatattgttcaaagaagtggcagctgaatgcatgaagaggtacattggcacaccttatgagggaattgtagacaccttagtttctctgattaatgtgttaacaaggtttacttggttccaggaagtggtgctatatggtaaaatatgtgagaccttcctaagatgctgcacagaatttaataggtcaggggtcaaactggttaagataaggcactgtaacattaacctatcagtcaaattgccatcaaataagaaagagaatatgttatgttgtctatatagtggaaacatggagctcttgcaaggacctttctatttgaacaggagacaagctgtccttggttcttcatacctttacattgtcattacactttacatacaagtgctgcagcagtacaggtgtctagaagttataaacagtgtgagtgaaaaaacattgcaagacattgaaaatcattccatgactctactagaagattcattcagggaaatcacttttgctcttgaaggtaggtttgaagaatcttataaaatacgaacctcgaggtgcagagccagtgggaattttctgaacaggagcagtagagaccactttataagcgttgtttcaggcttgaacctagtttatggcttcctcataaaagataacttactagccaactctcagcaacagaacaaacaactacagatgcttcgttttggcatgcttgcagggcttagtaggcttgtttgtcctaatgagctaggaaagaaattttcaacgagctgtagaagaattgaagacaacattgcaaggctttacctgcagacatccatttactgttcagtcagggatgtggaggacaatgttaagcactggaaacaaagagatctatgtcctgaagtaaccattccatgctttacagtctatggaacctttgtcaacagcgatagacaactgatctttgacatttacaatgtgcatatatataataaagaaatggacaactttgatgaaggatgtatcagcgtcttggaagaaacagcagaaaggcacatgctttgggaactcgatctgatgaattcactttgttctgacgaaaaaaaagatactagaaccgcaagactattactaggctgcccaaatgtgaggaaagcagcaaacagagaagggaagaagctgttgaagttaaacagtgacacatccacagacacacagagcattgcttctgaagtgtcggacagaaggtcttatagttcaagtaagagtagaatccgtagtatatttggtagatacaactctcagaagaaaccatttgaattaaggtcaggtcttgaggttttcaatgatcctttcaatgattatcagcaagcaataacggacatttgccaattttctgagtacacaccaaacaaagaaagcattttgaaagactgtcttcaaatcatacgaaaaaaccctagccacacaatgggttcttttgagctgatccaggcaatctcagagttcggcatgagcaagtttcctcccgaaaatatagacaaagcaagaagggatccgaagaactgggttagcatctctgaagtaaccgaaacaacaagtatagttgcatcacctagaactcatatgatgctcaaggattgttttaaaattatactaggtactgagaataagaagatagtcaaaatgcttcgaggtaagctaaagaaactcggtgctatctcaacaaacatagagatcgggaaaagggattgcctagatctactcagcacagtagatgggctaacagaccagcagaaagaaaatattgtaaatgggatatttgagccctcaaagttatccttctaccattggaaggaattggtcaaaaaaaacattgatgaagttttacttactgaagatggaaatctgatcttctgctggctgaaaacaatctcctcttcagtcaaaggaagcctaaagaagagactcaaattcatgaatatacattctccagaattgatgccggaaaactgtctcttttctagtgaggaattcaatgagttaattaagttgaagaaactcctcctcaatgaacaacaagatgaacaggagctgaaacaagatcttttgatatcttcttggatcaagtgcataacagcttgcaaggattttgcaagcatcaatgacaagattcagaagttcatttaccacctgtctgaagagctatatgacataaggctgcagcatctggaactgtcaaagcttaagcaagagcaccctagtgtcagcttcacaaaagaagaagtcttaataaagcggctggagaaaaatttccttaagcagcataatttagagattatggaaactgtgaatcttgtattctttgcagccctctcagctccctggtgcttacactataaagcactagagtcttatttggtgagacatccagaaatacttgactgtggatctaaggaggactgcaaactcaccttgcttgatctgtcagtttctaagctcttggtttgtttgtatcaaaaagatgatgaggagctgataaatagctcaagtttgaaacttgggtttttagtgaaatatgttgtcaccttgttcacatccaatggtgaacctttttcactcagtctcaatgacgggggtttggatcttgatttacacaagactactgacgaaaagttactacatcaaacaaagatagtttttgctaaaattggtttatctgggaacagttatgactttatctggactacccaaatgatagcaaacagcaattttaacgtctgcaaaagattaacgggaaggagtactggggaaaggctccctagaagcgttagaagcaaggtcatatatgagatggtaaaattagtgggagaaacaggcatggcaatactacaacaattagcttttgcacaagcactaaattatgagcaccgcttctatgcggtcttagcacctaaagcgcaactaggaggagcaagagatttgttagtgcaagagactgggactaaagtcatgcatgcaaccactgaaatgtttagtagaaatcttttaaaaacaacatcagatgatggcctcacaaacccacatcttaaagaaacaatccttaatgtgggattagactgtcttgctaacatgcgaaatcttgacggtaagcccataagtgaaggtagtaacttggtcaatttctacaaagtcatatgtatctcgggtgataataccaagtggggcccgatacactgctgttctttcttttctggcatgatgcaacaggttctgaaaaatgtaccagattggtgttcattttataaattaacattcattaaaaacttatgtagacaggtagaaatacctgctggcagtattaagaagatcttaaatgttcttaggtatagattgtgcagcaagggaggtgtagaacaacatagtgaagaagatctgagaagactgttgacagataatttagacagttgggatggaaacgacacagttaagttcttagttacaacttatataagcaaaggactcatggcgttaaacagttacaatcatatgggtcagggtattcaccatgcaacatcttcggtgttaacttccctagctgctgtgctctttgaggagctggcaattttttatcttaagagaagcttaccccagacaacagtacatgttgaacatgccggtagttcagatgattacgcaaagtgtatagtggtgactggtatactatccaaagagctctactcccagtatgatgaaacattttggaaacacgcttgcagactcaaaaacttcacggccgcggtacaaagatgctgtcaaatgaaagatagtgccaaaaccttggtgagcgactgctttctcgagttttacagtgagtttatgatgggctacagagtaacccctgctgtaataaagttcatgtttactggactgataaacagctctgtgacctctcctcagagtttgatgcaagcatgccaagtttcatcccaacaagcaatgtataatagtgttcctcttgtcaccaacactgccttcaccctattaaggcagcaaattttctttaaccatgttgaagactttatcagaaggtatggtatactgactcttgggactttgtcaccctttggtaggttgttcgtaccaacctactctggattagtcagctcagcggttgctttagaagatgctgaagtcattgctagagcagcccaaacacttcaaatgaacagtgtgtcaatacagtcaagtagcttgaccacattagatagcctaggtcgtagtaggacaagttccacagctgaggatagcagcagtgtgagcgacacaactgctgcttcccatgactcaggatcatcatcctcaagcttctcttttgagctcaatagacccctgtctgaaactgaactacagttcattaaagcactaagtagtctcaagtcaacacaagcctgtgaagtgattcaaaatagaattacaggtctttattgcaacagcaacgaaggacctcttgataggcataatgtcatttacagcagcagaatggcagactcttgcgattggctaaaggatggtaaaaggagagggaatctagaactagcgaataggatccaatctgtactgtgtattctgatagcaggatattacaggtcatttggaggggaaggaaccgagaaacaggtaaaggcatcattgaatagagacgacaataaaatcatagaggatcctatgatacaactaattccagaaaagctgaggagagagttagaaaggttaggtgtttctagaatggaagtcgatgagctaatgccaagcattagtcctgatgacaccttagcccagcttgtagcgaaaaaactcattagcctcaatgtttcgacagaagaatactcagctgaggtatctagactcaaacaaacactgacagcccgaaatgttttgcacgggttagctggagggattaaggagctttcgcttccaatatatacaatattcatgaaatcttacttctttaaagacaatgttttcctgtcactaacagatagatggtctaccaagcacagtacaaactatcgtgatagttgtggcaaacaattaaaaggtagaataattaccaagtatactcactggttggacacttttctgggctgctctgtctccatcaacaggcatactactgttaaagagccctccttattcaatccgaacatcagatgtgtgaatctgatcacatttgaggacggcctgagagaactatcagtgatacagagtcaccttaaagtctttgaaaatgagttcaccaacttaaatcttcaattctctgatccgaacagacagaaacttagaatagttgagtctagacctgcagaatctgagctagaggcaaaccgtgcagtaattgtcaagaccaaattgttttcagcaactgaacaagttcgactatccaacaaccctgcagttgtcatgggctacctattggatgaatcagcaatttcagaagtcaagcctaccaaggttgacttctcaaatttacttaaagaccgcttcaaaataatgcaattttttccttcagtgttcactttgattaagatgctgacagatgaatcgtcagattcagaaaagagtggccttagtccagatttgcaacaagttgcaagatactcaaaccatttgaccttgctcagcagaatgattcaacaagcaaagccaaccgtgactgttttctacatgctaaaaggtaacttgatgaacacagagccaacagttgctgagcttgtcagctatggtataaaggaaggcagattttttaggctttccgacaccggagtcgatgcaagcacatactctgtaaaatattggaaaattcttcactgcatctctgccattggatgtttacctttgagtcaagcagacaaatcttcactacttatgagcttcttaaactggagggtcaacatggacattagaacatctgactgtccactatctagtcatgaagcaagtatactgagtgaatttgatggacaagttatcgccaacatacttgccagtgaattgagttctgtgaaacgagattctgaacgcgagggtctaactgatctccttgattatctaaactcaccaactgaattgttgaagaagaagccttacttagggacaacttgcaagttcaacacctggggagactcgaatagatctggaaagttcacatacagcagcagatctggagaatccattggaatcttcattgcagggaaattgcacatccatctctcatctgagtccgttgccttgttgtgtgaaactgaaagacaagtgctttcttggatgagtaagaggaggactgaggtaataactaaagaacagcatcaactgtttctaagtcttctcccacagtctcatgagtgtttacaaaagcacaaggacggtagtgcgctatcagtcatacctgatagcagcaacccccgattacttaagtttgtgcccctcaaaaaaggtctagcagtggtgaaaatcaaaaaacaaattttaacagtgaagaagcaggttgtgtttgatgcagagagcgagcctagactgcagtgggggcatggctgcttgtccattgtttatgacgaaactgatactcagaccacataccatgaaaatcttttgaaggtgaagcatcttgtagactgctctacagatagaaaaaagcttttgccccagtcagtgttttctgactccaaagttgtcctttcaaggatcaagttcaagacggagcttctcctcaactcattgacgctgctccactgtttcctaaaacatgctcctagtgatgccataatggaggtagagagcaaaagtagcttgctacacaagtacctcaaatcgggaggtgtcaggcaacggaacactgaagtgctcttcagagagaagttaaacaaggttgttataaaagacaatcttgagcaaggtgtggaagaggagattgagttttgcaacaacttgactaagactgtttcagagaacccattaccactcagctgttggtctgaagttcaaaattacattgaagacataggctttaacaatgtacttgttaacattgacagaaacacggtgaaaagtgaacttttatggaaatttacgttagacaccaatgtaagcaccacaagtactataaaagacgtgaggacattggtgtcctacgttagcactgaaaccatccctaagttcttgcttgcattcttactttatgaagaagtgttaatgaacttaatcaaccagtgtaaggcagtaaaagaactcatcaacagcacaggactctcagacttggaactggaaagcttactcactttatgtgctttctatttccaaagtgagtgcagtaagagagatggtcctagatgctcctttgcagcactattaagtctaatccatgaggattggcagaggataggtaaaaacattcttgttcgtgcaaacaatgaactaggtgatgtgtcactgaaggttaacattgtcctggtgcctctcaaggacatgtctaagccaaagtctgagagagtggtcatggctagaaggtcactaaatcatgctctatccttgatgtttctggacgagatgtcactacctgagctaaaatccttatccgtgaactgcaaaatggggaactttgaagggcaggagtgctttgagttcactattctgaaggacaatagcgcaagactagattacaacaagttgattgaccactgtgtggacatggaaaaaaagagggaagcggttagagcagtagaagatttaattttgatgttgacaggcagagcagtcaaacccagcgctgtaacacagtttgtacacggggacgagcagtgtcaagagcaaataagcttagatgatctgatggcaaacgacacggtaacagactttcctgatagggaagcagaagccctcaaaacaggaaatcttggctttaactgggactcagattgacccgggcatgctcgagctagcagatctttttccctctgccaaaaattatggggacatcatgaagccccttgagcatctgacttctggctaataaaggaaatttattttcattgcaatagtgtgttggaattttttgtgtctctcactcggaaggacatatgggagggcaaatcatttaaaacatcagaatgagtatttggtttagagtttggcaacatatgccatatgctggctgccatgaacaaaggtggctataaagaggtcatcagtatatgaaacagccccctgctgtccattccttattccatagaaaagccttgacttgaggttagattttttttatattttgttttgtgttatttttttctttaacatccctaaaattttccttacatgttttactagccagatttttcctcctctcctgactactcccagtcatagctgtccctcttctcttatgaagatccctcgacctgcagcccaagcttggcgtaatcatggtcatagctgtttcctgtgtgaaattgttatccgctcacaattccacacaacatacgagccggaagcataaagtgtaaagcctggggtgcctaatgagtgagctaactcacattaattgcgttgcgctcactgcccgctttccagtcgggaaacctgtcgtgccagcggatccgcatctcaattagtcagcaaccatagtcccgcccctaactccgcccatcccgcccctaactccgcccagttccgcccattctccgccccatggctgactaattttttttatttatgcagaggccgaggccgcctcggcctctgagctattccagaagtagtgaggaggcttttttggaggcctaggcttttgcaaaaagctaacttgtttattgcagcttataatggttacaaataaagcaatagcatcacaaatttcacaaataaagcatttttttcactgcattctagttgtggtttgtccaaactcatcaatgtatcttatcatgtctggatccgctgcattaatgaatcggccaacgcgcggggagaggcggtttgcgtattgggcgctcttccgcttcctcgctcactgactcgctgcgctcggtcgttcggctgcggcgagcggtatcagctcactcaaaggcggtaatacggttatccacagaatcaggggataacgcaggaaagaacatgtgagcaaaaggccagcaaaaggccaggaaccgtaaaaaggccgcgttgctggcgtttttccataggctccgcccccctgacgagcatcacaaaaatcgacgctcaagtcagaggtggcgaaacccgacaggactataaagataccaggcgtttccccctggaagctccctcgtgcgctctcctgttccgaccctgccgcttaccggatacctgtccgcctttctcccttcgggaagcgtggcgctttctcaatgctcacgctgtaggtatctcagttcggtgtaggtcgttcgctccaagctgggctgtgtgcacgaaccccccgttcagcccgaccgctgcgccttatccggtaactatcgtcttgagtccaacccggtaagacacgacttatcgccactggcagcagccactggtaacaggattagcagagcgaggtatgtaggcggtgctacagagttcttgaagtggtggcctaactacggctacactagaaggacagtatttggtatctgcgctctgctgaagccagttaccttcggaaaaagagttggtagctcttgatccggcaaacaaaccaccgctggtagcggtggtttttttgtttgcaagcagcagattacgcgcagaaaaaaaggatctcaagaagatcctttgatcttttctacggggtctgacgctcagtggaacgaaaactcacgttaagggattttggtcatgagattatcaaaaaggatcttcacctagatccttttaaattaaaaatgaagttttaaatcaatctaaagtatatatgagtaaacttggtctgacagttaccaatgcttaatcagtgaggcacctatctcagcgatctgtctatttcgttcatccatagttgcctgactccccgtcgtgtagataactacgatacgggagggcttaccatctggccccagtgctgcaatgataccgcgagacccacgctcaccggctccagatttatcagcaataaaccagccagccggaagggccgagcgcagaagtggtcctgcaactttatccgcctccatccagtctattaattgttgccgggaagctagagtaagtagttcgccagttaatagtttgcgcaacgttgttgccattgctacaggcatcgtggtgtcacgctcgtcgtttggtatggcttcattcagctccggttcccaacgatcaaggcgagttacatgatcccccatgttgtgcaaaaaagcggttagctccttcggtcctccgatcgttgtcagaagtaagttggccgcagtgttatcactcatggttatggcagcactgcataattctcttactgtcatgccatccgtaagatgcttttctgtgactggtgagtactcaaccaagtcattctgagaatagtgtatgcggcgaccgagttgctcttgcccggcgtcaatacgggataataccgcgccacatagcagaactttaaaagtgctcatcattggaaaacgttcttcggggcgaaaactctcaaggatcttaccgctgttgagatccagttcgatgtaacccactcgtgcacccaactgatcttcagcatcttttactttcaccagcgtttctgggtgagcaaaaacaggaaggcaaaatgccgcaaaaaagggaataagggcgacacggaaatgttgaatactcatactcttcctttttcaatattattgaagcatttatcagggttattgtctcatgagcggatacatatttgaatgtatttagaaaaataaacaaataggggttccgcgcacatttccccgaaaagtgccacctg

SEQ ID NO: 5 - DNA, 9772 bp, Artificial Sequence
  Synthetic construct (pC-GPC-Oman)
cgcaccatgcccgtcaatactatgcacaccctgctggtctatgctgtcttctgtctgcagctgtggagccctgggggaacacgaggcctgagcaatgagacccagcacaacgaaacaggaatcacccgggcccccgaggggtcccagggaccttctctgccagtgtccacagcatctccaatcatgagtgacccctcaattaccacactgtcagccagcacttccggcctggaagggagcggagatactaccccccctgccattacacaggggcccactctgcctgagacaactcccgaaccttccaccacaactggaaccaatgcttttagtacagctatcgcaaacgtctcaacacagactgtgaaggacaccccaacacccactgtgcagactagcccaccctccaccccagatgcctctacaattccccagggcacccaccatacagctagggggctgctgagtgtgaccgtcacaaaaccagaggaagtgcctactccaaccggccccgagcaggcttccatcgaaaccaatagctccagactggcaacttctaagaccccctctcctagtccaacagcccaggtgaccacagagaactcaaatccaaacactagcaggcagctggtcctgagcacccagccagctacatctagtcctgtgaccagcccagcacagctgaacttcgtccagtccgctactaccatcgcagtgcaggacgcacacccatcccctactaatcgatctaagcggaacctggagatggaagtgattctgaccctgtcccaggggctgcgcaaatactatggacgaatcctgaagctgctggacctgactctggaggaagataccgagggcctgctggaatggtgtaaacgaaatctggggctgacctgcgacgataacttctttcagaagcggatcgaggagttcttcctgacaggcgaggggcactttaacgaagtgctgcagttcaagacaccttctactctgagtccaactgaatcagctagcgtcggactgccaaccgtggagcctttcaaatcatactttgcaaagggattcctgtcaattgacagcggctactttagtgcaaagtgttatcccagagcctccaattctgggctgcagctgatcaacgtgacacagcatagcgcaaggatcgccgatactccaggacccaaaattactaatctgaagaccatcaattgcattaacctgaaagctctggtgttcaaggagcacagagagatcgaaattaacgtgctgctgcctcaggtggcagtcaatctgtccaactgtcacgtccatattaagagccatgtgtgcgattactccctggacatcgatggcaccgtgagactgcctagaatccaccatgagggcacattcattccagggacttacaagatcgtgatcgacaagaaaaataagcagaacgatcgctgtaatctggtcaccaactgcgtgatcaaaggacgagaggtccgaaagggacagagcgtgctgcggcagtatagaacagaaatccggattggaaaggcttcaagcggcagtcggagactgctgtccgaggaatctggagaggactgcatttcacggacccagctgctgagaacagagactgccgaaatccacggggacaattacggcgggccaggagataaaatcactatttgtaacggctctaccattgtggatcagaggctgggcagtgagctggggtgctataccatcaatcgcgtgaagagcttcaagctgtgtgaaaacagtgccaccggcaagtcatgcgagattgacaacacacctgtgaagtgtaaacaggggttctgcctgaaaatcacccaggagggacgcggccacgtgaagctgagtcgagattcagaggtggtcctggacgcctgtgattcctcttgcgaaatcatgattccaaaagggacaggagacatcctggtggattgctccggaggccagcagcacttcctgaaggacaatctgatcgatctgggatgtccaaacattcccctgctgggcaaaatggccatctacatttgccgcatgagcaaccatcctaagacaactatggctttcctgttttggttctcctttggctacgtcatcacttgcattctgtgtaaagtgatcttctacctgctgattgtggtcggcaccctggggaagaaattcaaacagtatcgggaactgaagccccagacctgcacaatctgtgagaccacacctgtgaatgctattgacgcagaaatgcacgatctgaattgttcctacaacatctgcccatattgtgccagtcggctgacctcagacggcctggctagacatgtgatgcagtgccccaagaggaaagagaagattgaggaaacagaactgtacctgaacctggagcgaatcccttgggtggtccggaaactgctgcaggtcagtgagtcaaccggggtggcactgaagagaagttcatggctgatcgtcctgctggtgctgctgacagtcagcctgtccccagtgcagtccgcacctatcggccacgggaaaaccattgaaacataccagactagggagggatatacctctatctgtctgtttgtcctgggctctatcctgttcattgtgagtcatctgatgaagggactggtggacagcgtgggcaattccttctttcctgggctgtccatttgcaaaacctgtagcatcggcagcatcaacggctttgagatcgaatcacacaagtgctactgtagcctgttctgctgtccatattgcagacattgttctgccgataaagagatccacaagctgcatctgtcaatttgcaagaaaaggaaagccgggagcaatgtcatgctggctgtgtgtaagcgaatgtgctttcgggcaacaatggaggtgagcaataaggccctgctgatccgctcagtgattaacactaccttcgtggtctgtatcctgattctggctgtctgcgtggtctctaccagtgcagtggagatggaaagcctgccagcaggcacatgggagagagaggaagacctgactaacttttgtcaccaggaatgccaagtgactgagaccgaatgcctgtgtccttacgaggcactggtgctgaggaagccactgttcctggattccatcgccaaaggcatgaagaatctgctgaactcaacaagcctggaaacttccctgtctatcgaggctccttggggggcaattaatgtccagagcacctttaagccaaccgtgtccacagccaacatcgctctgtcttggagcagcgtcgagcaccgcggcaacaagatcctggtgagcggccggagcgaatcaattatgaagctggaggaaaggactggaatcagctgggacctgggcgtggaggatgctagcgaatccaagctgctgaccgtgtccgtcatggacctgtctcagatgtacagtcccgtcttcgagtatctgtctggagaccgccaggtggaggaatggcccaaagccacatgtactggagattgccctgagcggtgcggctgtacttctagtacctgtctgcacaaggaatggccacatagcaggaattggcgctgtaacccaacctggtgctggggagtgggcacagggtgcacttgctgtggcctggacgtgaaggacctgttcaccgactacatgttcgtcaaatggaaggtggagtatatcaagactgaagcaattgtgtgtgtcgagctgacctcccaggaacggcagtgctctctgatcgaggccgggaccagattcaacctgggacctgtgaccatcacactgagcgagccacgcaatattcagcagaagctgcctccagaaatcgtgacactgcacccccgaattgaggaaggcttctttgatctgatgcatgtccagaaagtgctgtctgccagtaccgtgtgtaagctgcagtcctgcacacacggagtccctggcgacctgcaggtgtaccatattgggaatctgctgaaaggagataaggtcaacggccacctgatccataaggtggagccacactttaacacctcttggatgagttgggacggctgtgacctggattactattgcaatatgggggattggccctcttgcacttacaccggagtcacacagcacaaccatgccgctttcgtgaatctgctgaacatcgagaccgactacacaaagaacttccactttcatagcaagagagtgaccgctcacggggacacaccccagctggatctgaaagctaggcctaactacggagcaggcgagatcaccgtgctggtcgaggtggccgatatggaactgcatacaaagaaaatcgaaattagtggactgaagttcgcatcactgacatgcactgggtgttatgcctgctcaagcggaatctcttgcaaagtccgcattcacgtggacgagcccgatgaactgaccgtccatgtgaagagcgaggaccctgatatcgtggcagcctcctctagtctgatggcccggaagctggaatttggcactgacagcaccttcaaagcattttccgccatgccaaagacatctctgtgtttctacatcgtggagcgcgaatattgtaaatcatgcagcaaggaggacactcagaaatgcgtgaatgccaagctggaacggccccagagcatcctgattgagcacaaagggaccatcattggaaagcagaacgatacctgtacagccaaggctagctgctggctggagtcagtgaagagcttcttctacggactgaagaatatgctgtccgggatttttggaaacgtgttcatcggcattttcctgtttctggccccctttatcctgctgattctgttctttatgttcggctggagaatcctgttctgctttaaatgctgtaggcgcacaagagggctgtttaaatacaggcacctgaaggacgatgaggaaactggatataggaagatcattgagcgcctgaacaataagaaaggcaaaaacaagctgctggacggggaaagactggccgataggaaaattgctgagctgttctccactaagacccatatcggctgatgatttttccctctgccaaaaattatggggacatcatgaagccccttgagcatctgacttctggctaataaaggaaatttattttcattgcaatagtgtgttggaattttttgtgtctctcactcggaaggacatatgggagggcaaatcatttaaaacatcagaatgagtatttggtttagagtttggcaacatatgccatatgctggctgccatgaacaaaggtggctataaagaggtcatcagtatatgaaacagccccctgctgtccattccttattccatagaaaagccttgacttgaggttagattttttttatattttgttttgtgttatttttttctttaacatccctaaaattttccttacatgttttactagccagatttttcctcctctcctgactactcccagtcatagctgtccctcttctcttatgaagatccctcgacctgcagcccaagcttggcgtaatcatggtcatagctgtttcctgtgtgaaattgttatccgctcacaattccacacaacatacgagccggaagcataaagtgtaaagcctggggtgcctaatgagtgagctaactcacattaattgcgttgcgctcactgcccgctttccagtcgggaaacctgtcgtgccagcggatccgcatctcaattagtcagcaaccatagtcccgcccctaactccgcccatcccgcccctaactccgcccagttccgcccattctccgccccatggctgactaattttttttatttatgcagaggccgaggccgcctcggcctctgagctattccagaagtagtgaggaggcttttttggaggcctaggcttttgcaaaaagctaacttgtttattgcagcttataatggttacaaataaagcaatagcatcacaaatttcacaaataaagcatttttttcactgcattctagttgtggtttgtccaaactcatcaatgtatcttatcatgtctggatccgctgcattaatgaatcggccaacgcgcggggagaggcggtttgcgtattgggcgctcttccgcttcctcgctcactgactcgctgcgctcggtcgttcggctgcggcgagcggtatcagctcactcaaaggcggtaatacggttatccacagaatcaggggataacgcaggaaagaacatgtgagcaaaaggccagcaaaaggccaggaaccgtaaaaaggccgcgttgctggcgtttttccataggctccgcccccctgacgagcatcacaaaaatcgacgctcaagtcagaggtggcgaaacccgacaggactataaagataccaggcgtttccccctggaagctccctcgtgcgctctcctgttccgaccctgccgcttaccggatacctgtccgcctttctcccttcgggaagcgtggcgctttctcaatgctcacgctgtaggtatctcagttcggtgtaggtcgttcgctccaagctgggctgtgtgcacgaaccccccgttcagcccgaccgctgcgccttatccggtaactatcgtcttgagtccaacccggtaagacacgacttatcgccactggcagcagccactggtaacaggattagcagagcgaggtatgtaggcggtgctacagagttcttgaagtggtggcctaactacggctacactagaaggacagtatttggtatctgcgctctgctgaagccagttaccttcggaaaaagagttggtagctcttgatccggcaaacaaaccaccgctggtagcggtggtttttttgtttgcaagcagcagattacgcgcagaaaaaaaggatctcaagaagatcctttgatcttttctacggggtctgacgctcagtggaacgaaaactcacgttaagggattttggtcatgagattatcaaaaaggatcttcacctagatccttttaaattaaaaatgaagttttaaatcaatctaaagtatatatgagtaaacttggtctgacagttaccaatgcttaatcagtgaggcacctatctcagcgatctgtctatttcgttcatccatagttgcctgactccccgtcgtgtagataactacgatacgggagggcttaccatctggccccagtgctgcaatgataccgcgagacccacgctcaccggctccagatttatcagcaataaaccagccagccggaagggccgagcgcagaagtggtcctgcaactttatccgcctccatccagtctattaattgttgccgggaagctagagtaagtagttcgccagttaatagtttgcgcaacgttgttgccattgctacaggcatcgtggtgtcacgctcgtcgtttggtatggcttcattcagctccggttcccaacgatcaaggcgagttacatgatcccccatgttgtgcaaaaaagcggttagctccttcggtcctccgatcgttgtcagaagtaagttggccgcagtgttatcactcatggttatggcagcactgcataattctcttactgtcatgccatccgtaagatgcttttctgtgactggtgagtactcaaccaagtcattctgagaatagtgtatgcggcgaccgagttgctcttgcccggcgtcaatacgggataataccgcgccacatagcagaactttaaaagtgctcatcattggaaaacgttcttcggggcgaaaactctcaaggatcttaccgctgttgagatccagttcgatgtaacccactcgtgcacccaactgatcttcagcatcttttactttcaccagcgtttctgggtgagcaaaaacaggaaggcaaaatgccgcaaaaaagggaataagggcgacacggaaatgttgaatactcatactcttcctttttcaatattattgaagcatttatcagggttattgtctcatgagcggatacatatttgaatgtatttagaaaaataaacaaataggggttccgcgcacatttccccgaaaagtgccacctggtcgacattgattattgactagttattaatagtaatcaattacggggtcattagttcatagcccatatatggagttccgcgttacataacttacggtaaatggcccgcctggctgaccgcccaacgacccccgcccattgacgtcaataatgacgtatgttcccatagtaacgccaatagggactttccattgacgtcaatgggtggactatttacggtaaactgcccacttggcagtacatcaagtgtatcatatgccaagtacgccccctattgacgtcaatgacggtaaatggcccgcctggcattatgcccagtacatgaccttatgggactttcctacttggcagtacatctacgtattagtcatcgctattaccatgggtcgaggtgagccccacgttctgcttcactctccccatctcccccccctccccacccccaattttgtatttatttattttttaattattttgtgcagcgatgggggcgggggggggggggccgcgcgccagccggggcggggcggggcgaggggcggggcggggcgaggcggagaggtgcggcggcagccaatcagagcggcgcgctccgaaagtttccttttatggcgaggcggcggcggcggcggccctataaaaagcgaagcgcgcggcgggcgggagtcgctgcgttgccttcgccccgtgccccgctccgcgccgcctcgcgccgcccgccccggctctgactgaccgcgttactcccacaggtgagcgggcgggacggcccttctcctccgggctgtaattagcgcttggtttaatgacggctcgtttcttttctgtggctgcgtgaaagccttaaagggctccgggagggccctttgtgcgggggggagcggctcggggggtgcgtgcgtgtgtgtgtgcgtggggagcgccgcgtgcggcccgcgctgcccggcggctgtgagcgctgcgggcgcggcgcggggctttgtgcgctccgcgtgtgcgcgaggggagcgcggccgggggcggtgccccgcggtgcgggggggctgcgaggggaacaaaggctgcgtgcggggtgtgtgcgtgggggggtgagcagggggtgtgggcgcggcggtcgggctgtaacccccccctgcacccccctccccgagttgctgagcacggcccggcttcgggtgcggggctccgtgcggggcgtggcgcggggctcgccgtgccgggcggggggtggcggcaggtgggggtgccgggcggggcggggccgcctcgggccggggagggctcgggggaggggcgcggcggccccggagcgccggcggctgtcgaggcgcggcgagccgcagccattgccttttatggtaatcgtgcgagagggcgcagggacttcctttgtcccaaatctggcggagccgaaatctgggaggcgccgccgcaccccctctagcgggcgcgggcgaagcggtgcggcgccggcaggaaggaaatgggcggggagggccttcgtgcgtcgccgcgccgccgtccccttctccatctccagcctcggggctgccgcagggggacggctgccttcgggggggacggggcagggcggggttcggcttctggcgtgtgaccggcggctctagagcctctgctaaccatgttcatgccttcttctttttcctacagctcctgggcaacgtgctggttgttgtgctgtctcatcattttggcaaagaattc

SEQ ID NO: 6 - protein, 482 aa, Crimean-Congo hemorrhagic fever virus
MENKIEVNNKDEMNRWFEEFKKGNGLVDTFTNSYSFCESVPNLDRFVFQMASATDDAQKDSIYASALVEATKFCAPIYECAWVSSTGIVKKGLEWFEKNAGTIKSWDESYTELKVDVPKIEQLTGYQQAALKWRKDIGFRVNANTAALSNKVLAEYKVPGEIVMSVKEMLSDMIRRRNLILNRGGDENPRGPVSHEHVDWCREFVKGKYIMAFNPPWGDINKSGRSGIALVATGLAKLAETEGKGIFDEAKKTVEALNGYLDKHKDEVDRASADSMITNLLKHIAKAQELYKNSSALRAQSAQIDTAFSSYYWLYKAGVTPETFPTVSQFLFELGKQPRGTKKMKKALLSTPMKWGKKLYELFADDSFQQNRIYMHPAVLTAGRISEMGVCFGTIPVANPDDAAQGSGHTKSILNLRTNTETNNPCAKTIVKLFEVQKTGFNIQDMDIVASEHLLHQSLVGKQSPFQNAYNVKGNATSANII

SEQ ID NO: 7 - protein, 3961 aa, Crimean-Congo hemorrhagic fever virus
MGKPIPNPLLGLDSTMDFLRSLDWTQVIAGQYVSNPRFNISDYFEIVRQPGDGNCFYHSIAELTMPNKTDHSYHYIKRLTESAARKYYQEEPEARLVGLSLEDYLKRMLSDNEWGSTLEASMLAKEMGITIIIWTVAASDEVEAAGIKFGDGDVFTAVNLLHSGQTHFDALRILPQFETDTREALSLMDRVIAVDQLTSSSSDELQDYEDLALALTSAEESNRRSSLDEVTLSKKQAEILRQKASQLSKLVNKSQNIPTRVGRVLDCMFNCKLCVEISADTLILRPESKEKIGEIMSLRQLGHKLLTRDKQIKQEFSRMKLYVTKDLLDHLDVGGLLRAAFPGTGIERHMQLLHSEMILDICTVSLGVMLSTFLYGSNNKNKKKFITNCLLSTALSGKKVYKVLGNLGNELLYKAPRKALATVCSALFGKQINKLQNCFRTISPVSLLALRNLDFDCLSVQDYNGMIENMSKLDNTDVEFNHREIADLNQLTSRLITLRKEKDTDLLKQWFPESDLTRRSIRNAANAEEFVISEFFKKKDIMKFISTSGRAMSAGKIGNVLSYAHNLYLSKSSLNMTSEDISQLLIEIKRLYALQEDSEVEPIAIICDGIESNMKQLFAILPPDCARECEVLFDDIRNSPTHSTAWKHALRLKGTAYEGLFANCYGWQYIPEDIKPSLTMLIQTLFPDKFEDFLDRTQLHPEFRDLTPDFSLTQKVHFKRNQIPSVENVQISIDATLPESVEAVPVTERKMFPLPETPLSEVHSIERIMENFTRLMHGGRLSTKKRDGDPAEQGNQQSITEHESSSISAFKDYGERGIVEENHMKFSGEDQLETRQLLLVEVGFQTDIDGKIRTDHKKWKDILKLLELLGIKCSFIACADCSSTPPDRWWITEDRVRVLKNSVSFLFNKLSRNSPTEVTDIVVGAISTQKVRSYLKAGTATKTPVSTKDVLETWEKMKEHILNRPTGLTLPTSLEQAMRKGLVEGVVISKEGSESCINMLKENLDRITDEFERTKFKHELTQNITTSEKMLLSWLSEDIKSSRCGECLSNIKKAVDETANLSEKIELLAYNLQLTNHCSNCHPNGVNISNTSNVCKRCPKIEVVSHCENKGFEDSNECLTDLDRLVRLTLPGKTEKERRVKRNVEYLIKLMMSMSGIDCIKYPTGQLITHGRVSAKHNDGNLKDRSDDDQRLAEKIDTVRKELSESKLKDYSTYARGVISNSLKNLSRQGKSKCSVPRSWLEKVLFDLKVPTKDEEVLINIRNSLKARSEFVRNNDKLLIRSKEELKKCFDVQSFKLKKNKQPVPFQVDCILFKEVAAECMKRYIGTPYEGIVDTLVSLINVLTRFTWFQEVVLYGKICETFLRCCTEFNRSGVKLVKIRHCNINLSVKLPSNKKENMLCCLYSGNMELLQGPFYLNRRQAVLGSSYLYIVITLYIQVLQQYRCLEVINSVSEKTLQDIENHSMTLLEDSFREITFALEGRFEESYKIRTSRCRASGNFLNRSSRDHFISVVSGLNLVYGFLIKDNLLANSQQQNKQLQMLRFGMLAGLSRLVCPNELGKKFSTSCRRIEDNIARLYLQTSIYCSVRDVEDNVKHWKQRDLCPEVTIPCFTVYGTFVNSDRQLIFDIYNVHIYNKEMDNFDEGCISVLEETAERHMLWELDLMNSLCSDEKKDTRTARLLLGCPNVRKAANREGKKLLKLNSDTSTDTQSIASEVSDRRSYSSSKSRIRSIFGRYNSQKKPFELRSGLEVFNDPFNDYQQAITDICQFSEYTPNKESILKDCLQIIRKNPSHTMGSFELIQAISEFGMSKFPPENIDKARRDPKNWVSISEVTETTSIVASPRTHMMLKDCFKIILGTENKKIVKMLRGKLKKLGAISTNIEIGKRDCLDLLSTVDGLTDQQKENIVNGIFEPSKLSFYHWKELVKKNIDEVLLTEDGNLIFCWLKTISSSVKGSLKKRLKFMNIHSPELMPENCLFSSEEFNELIKLKKLLLNEQQDEQELKQDLLISSWIKCITACKDFASINDKIQKFIYHLSEELYDIRLQHLELSKLKQEHPSVSFTKEEVLIKRLEKNFLKQHNLEIMETVNLVFFAALSAPWCLHYKALESYLVRHPEILDCGSKEDCKLTLLDLSVSKLLVCLYQKDDEELINSSSLKLGFLVKYVVTLFTSNGEPFSLSLNDGGLDLDLHKTTDEKLLHQTKIVFAKIGLSGNSYDFIWTTQMIANSNFNVCKRLTGRSTGERLPRSVRSKVIYEMVKLVGETGMAILQQLAFAQALNYEHRFYAVLAPKAQLGGARDLLVQETGTKVMHATTEMFSRNLLKTTSDDGLTNPHLKETILNVGLDCLANMRNLDGKPISEGSNLVNFYKVICISGDNTKWGPIHCCSFFSGMMQQVLKNVPDWCSFYKLTFIKNLCRQVEIPAGSIKKILNVLRYRLCSKGGVEQHSEEDLRRLLTDNLDSWDGNDTVKFLVTTYISKGLMALNSYNHMGQGIHHATSSVLTSLAAVLFEELAIFYLKRSLPQTTVHVEHAGSSDDYAKCIVVTGILSKELYSQYDETFWKHACRLKNFTAAVQRCCQMKDSAKTLVSDCFLEFYSEFMMGYRVTPAVIKFMFTGLINSSVTSPQSLMQACQVSSQQAMYNSVPLVTNTAFTLLRQQIFFNHVEDFIRRYGILTLGTLSPFGRLFVPTYSGLVSSAVALEDAEVIARAAQTLQMNSVSIQSSSLTTLDSLGRSRTSSTAEDSSSVSDTTAASHDSGSSSSSFSFELNRPLSETELQFIKALSSLKSTQACEVIQNRITGLYCNSNEGPLDRHNVIYSSRMADSCDWLKDGKRRGNLELANRIQSVLCILIAGYYRSFGGEGTEKQVKASLNRDDNKIIEDPMIQLIPEKLRRELERLGVSRMEVDELMPSISPDDTLAQLVAKKLISLNVSTEEYSAEVSRLKQTLTARNVLHGLAGGIKELSLPIYTIFMKSYFFKDNVFLSLTDRWSTKHSTNYRDSCGKQLKGRIITKYTHWLDTFLGCSVSINRHTTVKEPSLFNPNIRCVNLITFEDGLRELSVIQSHLKVFENEFTNLNLQFSDPNRQKLRIVESRPAESELEANRAVIVKTKLFSATEQVRLSNNPAVVMGYLLDESAISEVKPTKVDFSNLLKDRFKIMQFFPSVFTLIKMLTDESSDSEKSGLSPDLQQVARYSNHLTLLSRMIQQAKPTVTVFYMLKGNLMNTEPTVAELVSYGIKEGRFFRLSDTGVDASTYSVKYWKILHCISAIGCLPLSQADKSSLLMSFLNWRVNMDIRTSDCPLSSHEASILSEFDGQVIANILASELSSVKRDSEREGLTDLLDYLNSPTELLKKKPYLGTTCKFNTWGDSNRSGKFTYSSRSGESIGIFIAGKLHIHLSSESVALLCETERQVLSWMSKRRTEVITKEQHQLFLSLLPQSHECLQKHKDGSALSVIPDSSNPRLLKFVPLKKGLAVVKIKKQILTVKKQVVFDAESEPRLQWGHGCLSIVYDETDTQTTYHENLLKVKHLVDCSTDRKKLLPQSVFSDSKVVLSRIKFKTELLLNSLTLLHCFLKHAPSDAIMEVESKSSLLHKYLKSGGVRQRNTEVLFREKLNKVVIKDNLEQGVEEEIEFCNNLTKTVSENPLPLSCWSEVQNYIEDIGFNNVLVNIDRNTVKSELLWKFTLDTNVSTTSTIKDVRTLVSYVSTETIPKFLLAFLLYEEVLMNLINQCKAVKELINSTGLSDLELESLLTLCAFYFQSECSKRDGPRCSFAALLSLIHEDWQRIGKNILVRANNELGDVSLKVNIVLVPLKDMSKPKSERVVMARRSLNHALSLMFLDEMSLPELKSLSVNCKMGNFEGQECFEFTILKDNSARLDYNKLIDHCVDMEKKREAVRAVEDLILMLTGRAVKPSAVTQFVHGDEQCQEQISLDDLMANDTVTDFPDREAEALKTGNLGFNWDSD

SEQ ID NO: 8 - protein, 3946 aa, Artificial Sequence
  Synthetic polypeptide
  MISC_FEATURE (13)..(13): Xaa = Ile, Arg, Glu or Lys
  MISC_FEATURE (16)..(16): Xaa =  Gln or Arg
  MISC_FEATURE (18)..(18): Xaa =  Val or Ile
  MISC_FEATURE (40)..(40): Xaa =  Cys, Ala, Ser or Arg
  MISC_FEATURE (77)..(77): Xaa =  Pro, Asp or Thr
  MISC_FEATURE (120)..(120): Xaa =  Thr or Leu
  MISC_FEATURE (128)..(128): Xaa =  Glu or Val
  MISC_FEATURE (129)..(129): Xaa =  Ala, Arg or Gly
MDFLRSLDWTQVXAGXYXSNPRFNISDYFEIVRQPGDGNXFYHSIAELTMPNKTDHSYHYIKRLTESAARKYYQEEXEARLVGLSLEDYLKRMLSDNEWGSTLEASMLAKEMGITIIIWXVAASDEVXXAGIKFGDGDVFTAVNLLHSGQTHFDALRILPQFETDTREALSLMDRVIAVDQLTSSSSDELQDYEDLALALTSAEESNRRSSLDEVTLSKKQAEILRQKASQLSKLVNKSQNIPTRVGRVLDCMFNCKLCVEISADTLILRPESKEKIGEIMSLRQLGHKLLTRDKQIKQEFSRMKLYVTKDLLDHLDVGGLLRAAFPGTGIERHMQLLHSEMILDICTVSLGVMLSTFLYGSNNKNKKKFITNCLLSTALSGKKVYKVLGNLGNELLYKAPRKALATVCSALFGKQINKLQNCFRTISPVSLLALRNLDFDCLSVQDYNGMIENMSKLDNTDVEFNHREIADLNQLTSRLITLRKEKDTDLLKQWFPESDLTRRSIRNAANAEEFVISEFFKKKDIMKFISTSGRAMSAGKIGNVLSYAHNLYLSKSSLNMTSEDISQLLIEIKRLYALQEDSEVEPIAIICDGIESNMKQLFAILPPDCARECEVLFDDIRNSPTHSTAWKHALRLKGTAYEGLFANCYGWQYIPEDIKPSLTMLIQTLFPDKFEDFLDRTQLHPEFRDLTPDFSLTQKVHFKRNQIPSVENVQISIDATLPESVEAVPVTERKMFPLPETPLSEVHSIERIMENFTRLMHGGRLSTKKRDGDPAEQGNQQSITEHESSSISAFKDYGERGIVEENHMKFSGEDQLETRQLLLVEVGFQTDIDGKIRTDHKKWKDILKLLELLGIKCSFIACADCSSTPPDRWWITEDRVRVLKNSVSFLFNKLSRNSPTEVTDIVVGAISTQKVRSYLKAGTATKTPVSTKDVLETWEKMKEHILNRPTGLTLPTSLEQAMRKGLVEGVVISKEGSESCINMLKENLDRITDEFERTKFKHELTQNITTSEKMLLSWLSEDIKSSRCGECLSNIKKAVDETANLSEKIELLAYNLQLTNHCSNCHPNGVNISNTSNVCKRCPKIEVVSHCENKGFEDSNECLTDLDRLVRLTLPGKTEKERRVKRNVEYLIKLMMSMSGIDCIKYPTGQLITHGRVSAKHNDGNLKDRSDDDQRLAEKIDTVRKELSESKLKDYSTYARGVISNSLKNLSRQGKSKCSVPRSWLEKVLFDLKVPTKDEEVLINIRNSLKARSEFVRNNDKLLIRSKEELKKCFDVQSFKLKKNKQPVPFQVDCILFKEVAAECMKRYIGTPYEGIVDTLVSLINVLTRFTWFQEVVLYGKICETFLRCCTEFNRSGVKLVKIRHCNINLSVKLPSNKKENMLCCLYSGNMELLQGPFYLNRRQAVLGSSYLYIVITLYIQVLQQYRCLEVINSVSEKTLQDIENHSMTLLEDSFREITFALEGRFEESYKIRTSRCRASGNFLNRSSRDHFISVVSGLNLVYGFLIKDNLLANSQQQNKQLQMLRFGMLAGLSRLVCPNELGKKFSTSCRRIEDNIARLYLQTSIYCSVRDVEDNVKHWKQRDLCPEVTIPCFTVYGTFVNSDRQLIFDIYNVHIYNKEMDNFDEGCISVLEETAERHMLWELDLMNSLCSDEKKDTRTARLLLGCPNVRKAANREGKKLLKLNSDTSTDTQSIASEVSDRRSYSSSKSRIRSIFGRYNSQKKPFELRSGLEVFNDPFNDYQQAITDICQFSEYTPNKESILKDCLQIIRKNPSHTMGSFELIQAISEFGMSKFPPENIDKARRDPKNWVSISEVTETTSIVASPRTHMMLKDCFKIILGTENKKIVKMLRGKLKKLGAISTNIEIGKRDCLDLLSTVDGLTDQQKENIVNGIFEPSKLSFYHWKELVKKNIDEVLLTEDGNLIFCWLKTISSSVKGSLKKRLKFMNIHSPELMPENCLFSSEEFNELIKLKKLLLNEQQDEQELKQDLLISSWIKCITACKDFASINDKIQKFIYHLSEELYDIRLQHLELSKLKQEHPSVSFTKEEVLIKRLEKNFLKQHNLEIMETVNLVFFAALSAPWCLHYKALESYLVRHPEILDCGSKEDCKLTLLDLSVSKLLVCLYQKDDEELINSSSLKLGFLVKYVVTLFTSNGEPFSLSLNDGGLDLDLHKTTDEKLLHQTKIVFAKIGLSGNSYDFIWTTQMIANSNFNVCKRLTGRSTGERLPRSVRSKVIYEMVKLVGETGMAILQQLAFAQALNYEHRFYAVLAPKAQLGGARDLLVQETGTKVMHATTEMFSRNLLKTTSDDGLTNPHLKETILNVGLDCLANMRNLDGKPISEGSNLVNFYKVICISGDNTKWGPIHCCSFFSGMMQQVLKNVPDWCSFYKLTFIKNLCRQVEIPAGSIKKILNVLRYRLCSKGGVEQHSEEDLRRLLTDNLDSWDGNDTVKFLVTTYISKGLMALNSYNHMGQGIHHATSSVLTSLAAVLFEELAIFYLKRSLPQTTVHVEHAGSSDDYAKCIVVTGILSKELYSQYDETFWKHACRLKNFTAAVQRCCQMKDSAKTLVSDCFLEFYSEFMMGYRVTPAVIKFMFTGLINSSVTSPQSLMQACQVSSQQAMYNSVPLVTNTAFTLLRQQIFFNHVEDFIRRYGILTLGTLSPFGRLFVPTYSGLVSSAVALEDAEVIARAAQTLQMNSVSIQSSSLTTLDSLGRSRTSSTAEDSSSVSDTTAASHDSGSSSSSFSFELNRPLSETELQFIKALSSLKSTQACEVIQNRITGLYCNSNEGPLDRHNVIYSSRMADSCDWLKDGKRRGNLELANRIQSVLCILIAGYYRSFGGEGTEKQVKASLNRDDNKIIEDPMIQLIPEKLRRELERLGVSRMEVDELMPSISPDDTLAQLVAKKLISLNVSTEEYSAEVSRLKQTLTARNVLHGLAGGIKELSLPIYTIFMKSYFFKDNVFLSLTDRWSTKHSTNYRDSCGKQLKGRIITKYTHWLDTFLGCSVSINRHTTVKEPSLFNPNIRCVNLITFEDGLRELSVIQSHLKVFENEFTNLNLQFSDPNRQKLRIVESRPAESELEANRAVIVKTKLFSATEQVRLSNNPAVVMGYLLDESAISEVKPTKVDFSNLLKDRFKIMQFFPSVFTLIKMLTDESSDSEKSGLSPDLQQVARYSNHLTLLSRMIQQAKPTVTVFYMLKGNLMNTEPTVAELVSYGIKEGRFFRLSDTGVDASTYSVKYWKILHCISAIGCLPLSQADKSSLLMSFLNWRVNMDIRTSDCPLSSHEASILSEFDGQVIANILASELSSVKRDSEREGLTDLLDYLNSPTELLKKKPYLGTTCKFNTWGDSNRSGKFTYSSRSGESIGIFIAGKLHIHLSSESVALLCETERQVLSWMSKRRTEVITKEQHQLFLSLLPQSHECLQKHKDGSALSVIPDSSNPRLLKFVPLKKGLAVVKIKKQILTVKKQVVFDAESEPRLQWGHGCLSIVYDETDTQTTYHENLLKVKHLVDCSTDRKKLLPQSVFSDSKVVLSRIKFKTELLLNSLTLLHCFLKHAPSDAIMEVESKSSLLHKYLKSGGVRQRNTEVLFREKLNKVVIKDNLEQGVEEEIEFCNNLTKTVSENPLPLSCWSEVQNYIEDIGFNNVLVNIDRNTVKSELLWKFTLDTNVSTTSTIKDVRTLVSYVSTETIPKFLLAFLLYEEVLMNLINQCKAVKELINSTGLSDLELESLLTLCAFYFQSECSKRDGPRCSFAALLSLIHEDWQRIGKNILVRANNELGDVSLKVNIVLVPLKDMSKPKSERVVMARRSLNHALSLMFLDEMSLPELKSLSVNCKMGNFEGQECFEFTILKDNSARLDYNKLIDHCVDMEKKREAVRAVEDLILMLTGRAVKPSAVTQFVHGDEQCQEQISLDDLMANDTVTDFPDREAEALKTGNLGFNWDSD

SEQ ID NO: 9 - protein, 1687 aa, Crimean-Congo hemorrhagic fever virus
MPVNTMHTLLVYAVFCLQLWSPGGTRGLSNETQHNETGITRAPEGSQGPSLPVSTASPIMSDPSITTLSASTSGLEGSGDTTPPAITQGPTLPETTPEPSTTTGTNAFSTAIANVSTQTVKDTPTPTVQTSPPSTPDASTIPQGTHHTARGLLSVTVTKPEEVPTPTGPEQASIETNSSRLATSKTPSPSPTAQVTTENSNPNTSRQLVLSTQPATSSPVTSPAQLNFVQSATTIAVQDAHPSPTNRSKRNLEMEVILTLSQGLRKYYGRILKLLDLTLEEDTEGLLEWCKRNLGLTCDDNFFQKRIEEFFLTGEGHFNEVLQFKTPSTLSPTESASVGLPTVEPFKSYFAKGFLSIDSGYFSAKCYPRASNSGLQLINVTQHSARIADTPGPKITNLKTINCINLKALVFKEHREIEINVLLPQVAVNLSNCHVHIKSHVCDYSLDIDGTVRLPRIHHEGTFIPGTYKIVIDKKNKQNDRCNLVTNCVIKGREVRKGQSVLRQYRTEIRIGKASSGSRRLLSEESGEDCISRTQLLRTETAEIHGDNYGGPGDKITICNGSTIVDQRLGSELGCYTINRVKSFKLCENSATGKSCEIDNTPVKCKQGFCLKITQEGRGHVKLSRDSEVVLDACDSSCEIMIPKGTGDILVDCSGGQQHFLKDNLIDLGCPNIPLLGKMAIYICRMSNHPKTTMAFLFWFSFGYVITCILCKVIFYLLIVVGTLGKKFKQYRELKPQTCTICETTPVNAIDAEMHDLNCSYNICPYCASRLTSDGLARHVMQCPKRKEKIEETELYLNLERIPWVVRKLLQVSESTGVALKRSSWLIVLLVLLTVSLSPVQSAPIGHGKTIETYQTREGYTSICLFVLGSILFIVSHLMKGLVDSVGNSFFPGLSICKTCSIGSINGFEIESHKCYCSLFCCPYCRHCSADKEIHKLHLSICKKRKAGSNVMLAVCKRMCFRATMEVSNKALLIRSVINTTFVVCILILAVCVVSTSAVEMESLPAGTWEREEDLTNFCHQECQVTETECLCPYEALVLRKPLFLDSIAKGMKNLLNSTSLETSLSIEAPWGAINVQSTFKPTVSTANIALSWSSVEHRGNKILVSGRSESIMKLEERTGISWDLGVEDASESKLLTVSVMDLSQMYSPVFEYLSGDRQVEEWPKATCTGDCPERCGCTSSTCLHKEWPHSRNWRCNPTWCWGVGTGCTCCGLDVKDLFTDYMFVKWKVEYIKTEAIVCVELTSQERQCSLIEAGTRFNLGPVTITLSEPRNIQQKLPPEIVTLHPRIEEGFFDLMHVQKVLSASTVCKLQSCTHGVPGDLQVYHIGNLLKGDKVNGHLIHKVEPHFNTSWMSWDGCDLDYYCNMGDWPSCTYTGVTQHNHAAFVNLLNIETDYTKNFHFHSKRVTAHGDTPQLDLKARPNYGAGEITVLVEVADMELHTKKIEISGLKFASLTCTGCYACSSGISCKVRIHVDEPDELTVHVKSEDPDIVAASSSLMARKLEFGTDSTFKAFSAMPKTSLCFYIVEREYCKSCSKEDTQKCVNAKLERPQSILIEHKGTIIGKQNDTCTAKASCWLESVKSFFYGLKNMLSGIFGNVFIGIFLFLAPFILLILFFMFGWRILFCFKCCRRTRGLFKYRHLKDDEETGYRKIIERLNNKKGKNKLLDGERLADRKIAELFSTKTHIG

SEQ ID NO: 10 - DNA, 5064 bp, Artificial Sequence
  Synthetic polynucleotide
atgcccgtcaatactatgcacaccctgctggtctatgctgtcttctgtctgcagctgtggagccctgggggaacacgaggcctgagcaatgagacccagcacaacgaaacaggaatcacccgggcccccgaggggtcccagggaccttctctgccagtgtccacagcatctccaatcatgagtgacccctcaattaccacactgtcagccagcacttccggcctggaagggagcggagatactaccccccctgccattacacaggggcccactctgcctgagacaactcccgaaccttccaccacaactggaaccaatgcttttagtacagctatcgcaaacgtctcaacacagactgtgaaggacaccccaacacccactgtgcagactagcccaccctccaccccagatgcctctacaattccccagggcacccaccatacagctagggggctgctgagtgtgaccgtcacaaaaccagaggaagtgcctactccaaccggccccgagcaggcttccatcgaaaccaatagctccagactggcaacttctaagaccccctctcctagtccaacagcccaggtgaccacagagaactcaaatccaaacactagcaggcagctggtcctgagcacccagccagctacatctagtcctgtgaccagcccagcacagctgaacttcgtccagtccgctactaccatcgcagtgcaggacgcacacccatcccctactaatcgatctaagcggaacctggagatggaagtgattctgaccctgtcccaggggctgcgcaaatactatggacgaatcctgaagctgctggacctgactctggaggaagataccgagggcctgctggaatggtgtaaacgaaatctggggctgacctgcgacgataacttctttcagaagcggatcgaggagttcttcctgacaggcgaggggcactttaacgaagtgctgcagttcaagacaccttctactctgagtccaactgaatcagctagcgtcggactgccaaccgtggagcctttcaaatcatactttgcaaagggattcctgtcaattgacagcggctactttagtgcaaagtgttatcccagagcctccaattctgggctgcagctgatcaacgtgacacagcatagcgcaaggatcgccgatactccaggacccaaaattactaatctgaagaccatcaattgcattaacctgaaagctctggtgttcaaggagcacagagagatcgaaattaacgtgctgctgcctcaggtggcagtcaatctgtccaactgtcacgtccatattaagagccatgtgtgcgattactccctggacatcgatggcaccgtgagactgcctagaatccaccatgagggcacattcattccagggacttacaagatcgtgatcgacaagaaaaataagcagaacgatcgctgtaatctggtcaccaactgcgtgatcaaaggacgagaggtccgaaagggacagagcgtgctgcggcagtatagaacagaaatccggattggaaaggcttcaagcggcagtcggagactgctgtccgaggaatctggagaggactgcatttcacggacccagctgctgagaacagagactgccgaaatccacggggacaattacggcgggccaggagataaaatcactatttgtaacggctctaccattgtggatcagaggctgggcagtgagctggggtgctataccatcaatcgcgtgaagagcttcaagctgtgtgaaaacagtgccaccggcaagtcatgcgagattgacaacacacctgtgaagtgtaaacaggggttctgcctgaaaatcacccaggagggacgcggccacgtgaagctgagtcgagattcagaggtggtcctggacgcctgtgattcctcttgcgaaatcatgattccaaaagggacaggagacatcctggtggattgctccggaggccagcagcacttcctgaaggacaatctgatcgatctgggatgtccaaacattcccctgctgggcaaaatggccatctacatttgccgcatgagcaaccatcctaagacaactatggctttcctgttttggttctcctttggctacgtcatcacttgcattctgtgtaaagtgatcttctacctgctgattgtggtcggcaccctggggaagaaattcaaacagtatcgggaactgaagccccagacctgcacaatctgtgagaccacacctgtgaatgctattgacgcagaaatgcacgatctgaattgttcctacaacatctgcccatattgtgccagtcggctgacctcagacggcctggctagacatgtgatgcagtgccccaagaggaaagagaagattgaggaaacagaactgtacctgaacctggagcgaatcccttgggtggtccggaaactgctgcaggtcagtgagtcaaccggggtggcactgaagagaagttcatggctgatcgtcctgctggtgctgctgacagtcagcctgtccccagtgcagtccgcacctatcggccacgggaaaaccattgaaacataccagactagggagggatatacctctatctgtctgtttgtcctgggctctatcctgttcattgtgagtcatctgatgaagggactggtggacagcgtgggcaattccttctttcctgggctgtccatttgcaaaacctgtagcatcggcagcatcaacggctttgagatcgaatcacacaagtgctactgtagcctgttctgctgtccatattgcagacattgttctgccgataaagagatccacaagctgcatctgtcaatttgcaagaaaaggaaagccgggagcaatgtcatgctggctgtgtgtaagcgaatgtgctttcgggcaacaatggaggtgagcaataaggccctgctgatccgctcagtgattaacactaccttcgtggtctgtatcctgattctggctgtctgcgtggtctctaccagtgcagtggagatggaaagcctgccagcaggcacatgggagagagaggaagacctgactaacttttgtcaccaggaatgccaagtgactgagaccgaatgcctgtgtccttacgaggcactggtgctgaggaagccactgttcctggattccatcgccaaaggcatgaagaatctgctgaactcaacaagcctggaaacttccctgtctatcgaggctccttggggggcaattaatgtccagagcacctttaagccaaccgtgtccacagccaacatcgctctgtcttggagcagcgtcgagcaccgcggcaacaagatcctggtgagcggccggagcgaatcaattatgaagctggaggaaaggactggaatcagctgggacctgggcgtggaggatgctagcgaatccaagctgctgaccgtgtccgtcatggacctgtctcagatgtacagtcccgtcttcgagtatctgtctggagaccgccaggtggaggaatggcccaaagccacatgtactggagattgccctgagcggtgcggctgtacttctagtacctgtctgcacaaggaatggccacatagcaggaattggcgctgtaacccaacctggtgctggggagtgggcacagggtgcacttgctgtggcctggacgtgaaggacctgttcaccgactacatgttcgtcaaatggaaggtggagtatatcaagactgaagcaattgtgtgtgtcgagctgacctcccaggaacggcagtgctctctgatcgaggccgggaccagattcaacctgggacctgtgaccatcacactgagcgagccacgcaatattcagcagaagctgcctccagaaatcgtgacactgcacccccgaattgaggaaggcttctttgatctgatgcatgtccagaaagtgctgtctgccagtaccgtgtgtaagctgcagtcctgcacacacggagtccctggcgacctgcaggtgtaccatattgggaatctgctgaaaggagataaggtcaacggccacctgatccataaggtggagccacactttaacacctcttggatgagttgggacggctgtgacctggattactattgcaatatgggggattggccctcttgcacttacaccggagtcacacagcacaaccatgccgctttcgtgaatctgctgaacatcgagaccgactacacaaagaacttccactttcatagcaagagagtgaccgctcacggggacacaccccagctggatctgaaagctaggcctaactacggagcaggcgagatcaccgtgctggtcgaggtggccgatatggaactgcatacaaagaaaatcgaaattagtggactgaagttcgcatcactgacatgcactgggtgttatgcctgctcaagcggaatctcttgcaaagtccgcattcacgtggacgagcccgatgaactgaccgtccatgtgaagagcgaggaccctgatatcgtggcagcctcctctagtctgatggcccggaagctggaatttggcactgacagcaccttcaaagcattttccgccatgccaaagacatctctgtgtttctacatcgtggagcgcgaatattgtaaatcatgcagcaaggaggacactcagaaatgcgtgaatgccaagctggaacggccccagagcatcctgattgagcacaaagggaccatcattggaaagcagaacgatacctgtacagccaaggctagctgctggctggagtcagtgaagagcttcttctacggactgaagaatatgctgtccgggatttttggaaacgtgttcatcggcattttcctgtttctggccccctttatcctgctgattctgttctttatgttcggctggagaatcctgttctgctttaaatgctgtaggcgcacaagagggctgtttaaatacaggcacctgaaggacgatgaggaaactggatataggaagatcattgagcgcctgaacaataagaaaggcaaaaacaagctgctggacggggaaagactggccgataggaaaattgctgagctgttctccactaagacccatatcggctga

SEQ ID NO: 11 - DNA, 23 bp, Artificial Sequence
  Primer
atgaacaggtggtttgaagagtt

SEQ ID NO: 12 - DNA, 17 bp, Artificial Sequence
  Primer
tggcactggccatctga

SEQ ID NO: 13 - DNA, 25 bp, Artificial Sequence
  Probe
tgtccaaattgggaacactctcgca

SEQ ID NO: 14 - DNA, 21 bp, Artificial Sequence
  Primer
tgatgatgctgccttaggatc

SEQ ID NO: 15 - DNA, 21 bp, Artificial Sequence
  Primer
tggagactgttaccaacaaga

SEQ ID NO: 16 - DNA, 24 bp, Artificial Sequence
  Probe
tgcagcaggtgctcagaggctaca

SEQ ID NO: 17 - DNA, 18 bp, Artificial Sequence
  Primer
ggctgagtgtggagcacc

SEQ ID NO: 18 - DNA, 25 bp, Artificial Sequence
  Primer
aacaggatttaacatacaggacatg

SEQ ID NO: 19 - DNA, 24 bp, Artificial Sequence
  Probe
tcccttgttggcaagcagtctcca

SEQ ID NO: 20 - DNA, 21 bp, Artificial Sequence
  Primer
atggagactgttaccaacaag

SEQ ID NO: 21 - DNA, 21 bp, Artificial Sequence
  Primer
tgatgatgctgccttaggatc

SEQ ID NO: 22 - DNA, 24 bp, Artificial Sequence
  Probe
tgcagcaggtgctcagaggctaca